European Patent Specification EP 4 014 982 B1, published August 20, 2025. Title: COMPOSITION FOR INDUCING PROLIFERATION OR ACCUMULATION OF REGULATORY T CELLS. Applicant: The University of Tokyo. The sequence listing filed with the application follows.

SEQUENCE LISTING (69 sequences)

SEQ ID NO: 1 - DNA, 23 bp, Artificial
  Artificially synthesized primer sequence
ggcaatagttccttcccagagtt

SEQ ID NO: 2 - DNA, 22 bp, Artificial
  Artificially synthesized primer sequence
gggtcgcatattgtggtacttg

SEQ ID NO: 3 - DNA, 23 bp, Artificial
  Artificially synthesized primer sequence
ccttttgtagccctgctcactct

SEQ ID NO: 4 - DNA, 21 bp, Artificial
  Artificially synthesized primer sequence
gggtcacctgtatggcttcag

SEQ ID NO: 5 - DNA, 21 bp, Artificial
  Artificially synthesized primer sequence
tcagtgcaagatctgcaagca

SEQ ID NO: 6 - DNA, 19 bp, Artificial
  Artificially synthesized primer sequence
acaccggaagccaaacaca

SEQ ID NO: 7 - DNA, 27 bp, Artificial
  Artificially synthesized primer sequence
gattttaataagctccaagaccaaggt

SEQ ID NO: 8 - DNA, 27 bp, Artificial
  Artificially synthesized primer sequence
cttctatgcagttgatgaagatgtcaa

SEQ ID NO: 9 - DNA, 21 bp, Artificial
  Artificially synthesized primer sequence
cctcgtcccgtagacaaaatg

SEQ ID NO: 10 - DNA, 20 bp, Artificial
  Artificially synthesized primer sequence
tctccactttgccactgcaa

SEQ ID NO: 11 - DNA, 20 bp, Artificial
  Artificially synthesized primer sequence
ggacattgtctttgatggca

SEQ ID NO: 12 - DNA, 20 bp, Artificial
  Artificially synthesized primer sequence
cttgtcacgtggtgtcactg

SEQ ID NO: 13 - DNA, 20 bp, Artificial
  Artificially synthesized primer sequence
tctctggacgtcaaatgtgg

SEQ ID NO: 14 - DNA, 19 bp, Artificial
  Artificially synthesized primer sequence
gctgaacagcagagccttc

SEQ ID NO: 15 - DNA, 20 bp, Artificial
  Artificially synthesized primer sequence
aggtctggatcactccaagg

SEQ ID NO: 16 - DNA, 19 bp, Artificial
  Artificially synthesized primer sequence
tcgcctggaccataaagaa

SEQ ID NO: 17 - DNA, 20 bp, Artificial
  Artificially synthesized primer sequence
agaggatgcgtgactttgtg

SEQ ID NO: 18 - DNA, 20 bp, Artificial
  Artificially synthesized primer sequence
atacagcagaccttctggca

SEQ ID NO: 19 - DNA, 20 bp, Artificial
  Artificially synthesized primer sequence
agagtttgatcmtggctcag

SEQ ID NO: 20 - DNA, 16 bp, Artificial
  Artificially synthesized primer sequence
attaccgcggckgctg

SEQ ID NO: 21 - DNA, 1460 bp, Clostridium leptum
  rRNA (1)..(1460): 16S rRNA coding gene sequence of Clostridium strain 1
agagtttgatcctggctcaggatgaacgctggcggcgtgcttaacacatgcaagtcgaacgagaaccattggatcgaggattcgtccaagtgaaggtggggaaagtggcggacgggtgagtaacgcgtgagcaatctgccttggagtggggaataacggctggaaacagccgctaataccgcatgatacagctgggaggcatctccctggctgtcaaagatttatcgctctgagatgagctcgcgtctgattagctagttggcggggtaacggcccaccaaggcgacgatcagtagccggactgagaggttggccggccacattgggactgagacacggcccagactcctacgggaggcagcagtggggaatattgggcaatgggcgcaagcctgacccagcaacgccgcgtgaaggaagaaggctttcgggttgtaaacttcttttgtcagggacgaagcaagtgacggtacctgacacggctactacggtcagcagcgcgtatacgtaggtgccagcgtatccggaattacctgggttaaggcgtgttagccggactgcagtcagatgtgaatcacgggctcaacttgtgctgcattggaactgtagttctgagtactgagagcagacggaattctaggtagcggtgaatgcgtagatataggaggacacagtgcgaggcgtctgctgacagcaactgacgctgaggcgggaagcgtgggggagccaacaggattagatacctggtagttcacgcctggtaaaacgatggatactaggtgtggggggactgaccccctcgtggccgccagttaacaccaataaagtatcccacctgggagtacgatcgcaaggttgaaactcaaaggaattgacggggcccgcacaagcggtggagtatgtggtttaattcgaagcaacgcgaagaaccttaccagggcttgacatcccgaggaccggactagagatagtcttttctcttcggagacctcggtgacaggtggtgcatggttgtcgtcagctcgtgtcgtaagatgttgggttaagtcccgcaacgagcgcaacccttattgttagttgctacgcaagagcactctagcgagactgccgttgacaaaacggaggaaggtggggacgacgtcaaatcatcatgccccttatgtcctgggccacacacgtactacaatggtggtcaacagagggaagcaataccgcgaggtggagcaaatccctaaaagccatcccagttcggatcgcaggctgcaacccgcctgcgtgaagttggaatcgctagtaatcgcggatcagcatgccgcggtgaatacgttcccgggccttgtacacaccgcccgtcacaccatgagagtcgggaacacccgaagtccgtagcctaaccgcaagggggggcgcggccgaaggtgggttcgataattggggtgaagtcgtaacaaggtagccgt

SEQ ID NO: 22 - DNA, 1485 bp, Clostridium leptum
  rRNA (1)..(1485): 16S rRNA coding gene sequence of Clostridium strain 2
agagtttgatcctggctcaggatgaacgctggcggcgtgcttaacacatgcaagtcgaacggagcacccctgaaggagttttcggacaacggaagggactgcttagtggcggacgggtgagtaacgcgtgaggaacctgccttggagtggggaataacagctggaaacagctgctaataccgcataatatatctgggccgcatggctctggatatcaaagatttatcgctctgagatggactcgcgtctgattagctagttggcggggtaacggcccaccaaggcgacgatcagtagccggactgagaggttggccggccacattgggactgagacacggcccagactcctacgggaggcagcagtggggaatattgggcaatgggcgcaagcctgacccagcaacgccgcgtgaaggaagaaggctttcgggttgtaaacttcttttgtcagggacgaagcaagtgacggtacctgacgaataagccacggctaactacgtgccagcagccgcggtaatacgtaggtggcaagcgttatccggatttactgggtgtaaagggcgtgtaggcgggactgcaagtcagatgtgaaaaccacgggctcaacctgtgggcctgcatttgaaactgtagttcttgagtactggagaggcagacggaattctagttgtagcgtgaaatgcgtagatatagaagaacacagttgcggagccggtctgcaactgacgctgagcgcgaaagcgtggggagcaaacaggattagataccctggtagtccacgctgtaaacgatggattactaggtgtggggggactgaccccctccgtgccgcagttaacacaataagtatcccacctggggagtacgatcgcaaggttgaaactcaaaaggaattgacgggggcccgcacaagcggtggagtatgtggtttaaattcgaagcaacgcgaagaaccttaccagggcttgacatcccggtgaccgtcctagagataggattttcccttcggggacactggagacaggtggtgcatggttgtcgtcagctcgtgtcgtgagatgttgggttaagtcccgcaacgagcgcaacccttattgttagttgctacgcaagagcactctagcgagactgccgttgacaaaacggaggaaggtggggacgacgtcaaatcatcatgccccttatgtcctgggccacacacgtactacaatggtggtcaacagagggaagcaaagccgcgaggtggagcaaatccctaaaagccatcccagttcggatcgcaggctgcaacccgcctgcgtgaagttggaatcgctagtaatcgcggatcagaatgccgcggtgaatacgttcccgggccttgtacacaccgcccgtcacaccatgagagtcgggaacacccgaagtccgtagcctaaccgcaaggggggcgcggccgaaggtgggttcgataattggggtgaagtcgtaacaaggtagccgt

SEQ ID NO: 23 - DNA, 1491 bp, Clostridium leptum
  rRNA (1)..(1491): 16S rRNA coding gene sequence of Clostridium strain 3
agagtttgatcctggctcaggacgaacgctggcggcgtgcttaacacatgcaagtcgaacggagcaccttcgaaagagacttcggtcaatggaaaagaatgcttagtggcggacgggtgagtaacgcgtgaggaacctgcctttcagtgggggacaacagttggaaacgactgctaataccgcataacgtacgggtatcgcatggtatctgtaccaaagatttatcgctgagagatggcctcgcgtctgattagctagttggtagggtaacggcctaccaaggcgacgatcagtagccggactgagaggttggccggccacattgggactgagatacggcccagactcctacgggaggcagcagtggggaatattgggcaatgggcgaaagcctgacccagcaacgccgcgtgaaggaagaaggctttcgggttgtaaacttcttttgacggggaagagcagaagacggtacctgtcgaataagccacggctaactacgtgccagcagccgcggtaatacgtaggtggcaagcgttgtccggatttactgggtgtaaagggcgtgtagccgggctgacaagtcagatgtgaaatccgggggctcaacccccgaactgcatttgaaactgttggtcttgagtatcggagaggcaggcggaattcctagtgtagcggtgaaatgcgtagatattagggggaacaccagtggcgaagcggcctgctggacgacaactgacggtgaggcgcgaaagcgtggggagcaaacaggattagataccctggtagtccacgctgtaaacgatggatactaggtgtgcggggactgacccctgcgtgccgcagctaacgcaataagtatcccacctggggagtacgatcgcaaggttgaaactcaaaggaattgacgggggcccgcacaagcggtggattatgtggtttaattcgatgcaacgcgaagaaccttaccagggcttgacatcctactaacgaagtagagatacattaggtacccttcgggggaagtagagacaggtggtgcatggttgtcgtcagctcgtgtcgtgagatgttgggttaagtcccgcaacgagcgcaacccttattgttagttgctacgcaagagcactctagcgagactgccgttgacaaaacggaggaaggtggggacgacgtcaaatcatcatgccccttatgtcctgggctacacacgtaatacaatggcggtcaacagagggatgcaaaaccgcgaggtggagcgaacccctaaaagccgtcccagttcagatcgcagtctgcaacccgactgcgtgaagtcggaatcgctagtaatcgcggatcagcatgccgcggtgaatacgttcccgggccttgtacacaccgcccgtcacaccatgagagtcgggaacacccgaagtccgtagcctaaccgcaaggagggcgcggccgaaggtgggttcgataattggggtgaagtcgtaacaaggtagccgt

SEQ ID NO: 24 - DNA, 1491 bp, Clostridium coccoides
  rRNA (1)..(1491): 16S rRNA coding gene sequence of Clostridium strain 4
agagtttgatcctggctcaggatgaacgctggcggcgtgcctaacacatgcaagtcgaacgggtgtacggggaggaaggcttcggccggaaaacctgtgcatgagtggcggacgggtgagtaacgcgtgggcaacctggcctgtacagggggataacacttagaaataggtgctaataccgcataacgggggaagccgcatggcttttccctgaaaactccggtggtacaggatgggcccgcgtctgattagccagttggcagggtaacggcctaccaaagcgacgatcagtagccggcctgagagggcggacggccacactgggactgagacacggcccagactcctacgggaggcagcagtgggggatattgcacaatggggggaaaccctgatgcagcgacgccgcgtgagtgaagaagtatttcggtatgtaaagctctatcagcagggaagaaaatgacggtacctgactaagaagccccggctaactacgtgccagcagccgcggtaatacgtagggggcaagcgttatccggatttactgggtgtaaagggagcgtagacggcagcgcaagtctgagtgaaatcccatggcttaaccatggaactgctttggaaactgtgcagctggagtgcaggagagtaagcggaattcctagtgtagcgtgaaatgcgtagattataggaggaacaccagtggcgaaggcggctaactgaactgtaactgacgttgaggctcgaaagcgtggggagcaaacaggattagataccctggtagtccacgccgtaaacgatgattactaggtgttgggggaccaaggtcttcggtgccggcgcaaacgcattaagtaatccacctggggagtacgttcgcaagaatgaaactcaaaggaattgacggggacccgcacaagcggtggagcatgtggtttaattcgaagcaacgcgaagaaccttacctggtcttgacatcccgatgacgagtgagcaaagtcactttcccttcggggcattggagacaggtggtgcatggttgtcgtcagctcgtgtcgtgagatgttgggttaagtcccgcaacgagcgcaacccctatttccagtagccagcaggtagagctgggcactctggagagactgcccgggataaccgggaggaaggcggggatgacgtcaaatcatcatgccccttatgatcagggctacacacgtgctacaatggcgtaaacaaagggaagcgagacggtgacgttgagcaaatcccaaaaataacgtcccagttcggattgtagtctgcaactcgactacatgaagctggaatcgctagtaatcgcgaatcagaatgtcgcggtgaatacgttcccgggtcttgtacacaccgcccgtcacaccatgggagtcggaaatgcccgaagtcagtgacctaaccgaaaggaaggagctgccgaaggtggagccggtaactggggtgaagtcgtaacaaggtagccgt

SEQ ID NO: 25 - DNA, 1467 bp, Clostridium leptum
  rRNA (1)..(1467): 16S rRNA coding gene sequence of Clostridium strain 5
agagtttgatcctggctcaggacgaacgctggcggcacgcctaacacatgcaagtcgaacggagtgaagatgctcgcatctgaacttagtggcggacgggtgagtaacacgtgagcaacctgcctttcagagggggattacgtttggaaacgaacgctaataccgcataaaatatcggagtcgcatggcactgatatcaaaggagcaatccgctgaaagatgggctcgcgtccgattaggcagttggcggggtatcggcccaccaaaccgacaatcggtagccggactgagaggttgaacggccacattgggactgagacgcggcccagactcctacgggaggcagcagtgggggatattgcacaatgggggaaaccctgatgcagcgatgccgcgtgaatgaagacggccttcgggttgtaaagttctgtcgcaggggacgaaaatgacggtaccctgcaagaaagctccggctaactacgtgccagcagccgcggtaatacgtagggagcaagcgttgtccggaattactgggtgtaaagggagcgtaggcgggaggataagttgaatgtgaaatctatgggctcaacccatagctgcgttcaaactgttcttcttgagtgaagtagaggcaggcggaattcctagtgtagcggtgaaatgcgtagatattaggaggacaccagtggcgaaggcgggctgctgggctttactgacgctgaggctcgaaagcgtgggtagcaaacaggattagataccctggtagtccacgcggtaaacgatgattactaggtgtgggtggactgaccccatccgtgccggagttaacacaataagtaatccacctggggagtacggccgcaaggttgaaactcaaaggaattgacgggggcccgcacaagcagtggagtatgtggtttaattcgacgcaacgcgaagaaccttaccaggtcttgacatcgagtgacggacatagagatatgtctttccttcgggacacgaagacaggtggtgcatggttgtcgtcagctcgtgtcgtgagatgttgggttaagtcccgcaacgagcgcaacccttaccattagttgctacgcaagagcactctaatgggactgccgttgacaaaacggaggaaggtggggatgacgtcaaatcatcatgccccttatgacctgggcgacacacgtactacaatggcggtcaacagagggaggcaaagccgcgaggcagagcaaacccctaaaagccgtctcagttcggattgcaggctgcaactcgcctgcatgaagtcggaattgctagtaatcgcggatcagcatgccgcggtgaatacgttcccgggccttgtacacaccgcccgtcacaccatgagagccggtaacacccgaagtcaatagtctaaccgcaaggaggacattgccgaaggtgggattggtaattggggtgaagtcgtaacaaggtagccgt

SEQ ID NO: 26 - DNA, 1474 bp, Clostridium coccoides
  rRNA (1)..(1474): 16S rRNA coding gene sequence of Clostridium strain 6
agagtttgatcatggctcaggatgaacgctggcggcgtgcctaacacatgcaagtcgaacgggtgtacgggaaggaaggcttcggccggaaaacctgtgcatgagtggcggacgggtgagtaacgcgtgggcaacctggcctgtacagggggataacacttagaaataggtgctaataccgcataacgggggaagccgcatggcttttccctgaaaactccggtggtacaggatgggcccgcgtctgattagccagttggcagggtaacggcctaccaaagcgacgatcagtagccggcctgagagggcggacggccacactgggactgagacacggcccagactcctacgggaggcagcagtgggggatattgcacaatggggggaaccctgatgcagcgacgccgcgtgggtgaagaagcgcctcggcgcgtaaagccctgtcagcagggaagaaaatgacggtacctgaagaagaagccccggctaactacgtgccagcagccgcggtaatacgtaggggggcaagcgttatccggatttactgggtgtaaagggggcgcagacggcgatgcaagccaggagtgaaagcccggggcccaaccccgggactgctcttgggaactgcgtggctggagtgcagagggcagcggaattcctggtgaaatgcgtagatatcagaagacacggtgcgaggcggcctgctgactgcactgacgttgagccgaagcgtggggagcaaacaggattagataccgtggtagtcacgccgtaaacgatgattactaggtgtcggggagcagagactgcccggtgccgcagccaacgcattaagtaatccacctggggagtacgttcgcaagaatgaaactcaaaggaattgacggggacccgcacaagcggtggagcatgtggtttaattcgaagcaacgcgaagaaccttacctggtcttgacatcccgatgacgagtgagcaaagtcactttcccttcggggcattggagacaggtggtgcatggttgtcgtcagctcgtgtcgtgagatgttgggttaagtcccgcaacgagcgcaacccctatttccagtagccagcaggtagagctgggcactctggagagactgcccgggataaccgggaggaaggcggggatgacgtcaaatcatcatgccccttatgatcagggctacacacgtgctacaatggcgtaaacaaagggaagcgagacggtgacgttaagcaaatcccaaaaataacgtcccagttcggattgtagtctgcaactcgactacatgaagctggaatcgctagtaatcgcgaatcagaatgtcgcggtgaatacgttcccgggtcttgtacacaccgcccgtcacaccatgggagtcggaaatgcccgaagtcagtgacctaaccgaaaggaaggagctgccgaaggtggagccggtaactggggtgaagtcgtaacaaggtagccgt

SEQ ID NO: 27 - DNA, 1484 bp, Clostridium leptum
  rRNA (1)..(1484): 16S rRNA coding gene sequence of Clostridium strain 7
agagtttgatcctggctcaggatgaacgctggcggcgtgcttaacacatgcaagtcgaacgagaatccagtgaaggagttttcggacaacggatctggaggaaagtggcggacgggtgagtaacgcgtgagcaatctgccttggagtggggaataacggttggaaacagccgctaataccgcatgatgcgtctgggaggcatctctctggacgccaaagatttatcgctctgagatgagctcgcgtctgattagcttgttggcggggtaaaggcccaccaaggcgacgatcagtagccggactgagaggttggccggccacattgggactgagacacggcccagactcctacgggaggcagcagtggggaatattgggcaatgggcgcaagcctgacccagcaacgccgcgtgaaggaagaaggctttcgggttgtaaacttcttttctgagggacgaagaaagtgacggtacctcaggaataagccacggctaactacgtgccagcagccgcggtaatacgtaggtggcaagcgttatccggatttattgggtgtaaagggcgtgtaggcgggaaagcaagtcagatgtgaaaactcagggctcaaccctgagcctgcatttgaaactgtttttcttgagtgctggagaggcaatcggaattccgtgtgtagcggtgaaatgcgtagatatacggaggacaccagtggcgagcggattgctggacagtactgacgctgaagcgcgaaagcgtgggagcaaacagatagatacctggtagtcacgcgtaaacgatggatactaggtgtggggggactgaccccctccgtgccgcagctaacgcaataagtatcccacctggggagtacgatcgcaaggttgaaactcaaaggaattgacgggggcccgcacaagcggtggagtatgtggtttaattcgaagcaacgcgaagaaccttaccagggcttgacatcctgctaacgaaccagagatggattaggtgcccttcggggaaagcagagacaggtggtgcatggttgtcgtcagctcgtgtcgtgagatgttgggttaagtcccgcaacgagcgcaacccttattgttagttgctacgcaagagcactctagcgagactgccgttgacaaaacggaggaaggtggggacgacgtcaaatcatcatgccccttacgtcctgggccacacacgtactacaatggcggccaacaaagagaggcaagaccgcgaggtggagcaaatctcaaaaagccgtcccagttcggatcgcaggctgcaacccgcctgcgtgaagttggaatcgctagtaatcgcggatcagcatgccgcggtgaatacgttcccgggccttgtacacaccgcccgtcacaccatgagagtcgggaacacccgaagtccgtagcctaaccgcaaggggggcgcggccgaaggtgggttcgataattggggtgaagtcgtaacaaggtagccgt

SEQ ID NO: 28 - DNA, 1483 bp, Clostridium leptum
  rRNA (1)..(1483): 16S rRNA coding gene sequence of Clostridium strain 8
agagtttgatcctggctcaggacgaacgctggcggcgtgcttaacacatgcaagtcgaacggagcacccctgaaggagttttcggacaacggatgggaatgcttagtggcggactggtgagtaacgcgtgaggaacctgccttccagagggggacaacagttggaaacgactgctaataccgcatgatgcgttggagccgcatgactccgacgtcaaagatttatcgctggaagatggcctcgcgtctgattagctagttggtgaggtaacggcccaccaaggcgacgatcagtagccggactgagaggttggccggccacattgggactgagatacggcccagactcctacgggaggcagcagtggggaatattgggcaatggacgcaagtctgacccagcaacgccgcgtgaaggaagaaggctttcgggttgtaaacttcttttaagggggaagagcagaagacggtaccccttgaataagccacggctaactacgtgccagcagccgcggtaatacgtaggtggcaagcgttgtccggatttactgggtgtaaagggcgtgcagccggagagacaagtcagatgtgaaatccacgggctcaacccgtgaactgcatttgaaactgtttcctttgagtgtcggagaggtaatcgggattccttgtgtagcggtgaatgcgtagatatagagaccacagtgccgacgccgaatactgacgatactgacggtgagcgcgaaagcgtggggagcaaacaggattagataccctggtagtccacgctgtaaacgatcgatactaggtgtgcggggactgacccctgcgtgccggagttaacacaataagtatcgcacctggggagtacgatcgcaaggttgaaactcaaaggaattgacgggggcccgcacaagcggtggattatgtggtttaattcgaagcaacgcgaagaaccttaccagggcttgacatcctgctaacgaagtagagatacattaggtgcccttcggggaaagcagagacaggtggtgcatggttgtcgtcagctcgtgtcgtgagatgttgggttaagtcccgcaacgagcgcaacccctattgttagttgctacgcaagagcactctagcgagactgccgttgacaaaacggaggaaggcggggacgacgtcaaatcatcatgccccttatgtcctgggctacacacgtaatacaatggcggttaacaaagggatgcaaagccgcgaggcagagcgaaccccaaaaagccgtcccagttcggatcgcaggctgcaacccgcctgcgtgaagtcggaatcgctagtaatcgcggatcagcatgccgcggtgaatacgttcccgggccttgtacacaccgcccgtcacaccatgagagtcgggaacacccgaagtccgtagcctaaccgcaaggagggcgcggccgaaggtgggttcgataattggggtgaagtcgtaacaaggtagccgt

SEQ ID NO: 29 - DNA, 1480 bp, Clostridium coccoides
  rRNA (1)..(1480): 16S rRNA coding gene sequence of Clostridium strain 9
ggagtttgatcctggctcaggatgaacgctggcggcgtgcttaacacatgcaagtcgaacgggctcatattgaaacctagtgatgtatgagttagtggcggacgggtgagtaacgcgtggagaacctgccgtatactgggggataacacttagaaataggtgctaataccgcataagcgcacagcttcgcatgaagcagtgtgaaaaactccggtggtatacgatggatccgcgtctgattagctggttggcggggtaacagcccaccaaggcgacgatcagtagccggcctgagagggtgaacggccacattgggactgagacacggcccaaactcctacgggaggcagcagtggggaatattgcacaatgggggaaaccctgatgcagcgacgccgcgtgagtgaagaagtatttcggtatgtaaagctctatcagcagggaagaaatactgaccttacggtcagcagacggtacctgactaagaagccccgggctaactacgtgccagcagccgcggtaatacgtaggggcaagcgttatccggatttactgggtgtaaagggggcgcagacggcgatgcaagccaggagtgaaagccggggcccaaccccgggactgctcttggactgcgtggctggagtgcagagggcagcgaattcctgtgtagcgtgaatgcgtagattcagaggacacgtgcgagcgcctgctgactgcactgacgtgagcccgaagcgtggggagcaaacaggattagatacctggtagtccacgccgtaaacgatgattactaggtgtcggggagcagagactgcccggtgccgcagccaacgcattaagtaatccacctggggagtacgttcgcaagaatgaaactcaaaggaattgacggggacccgcacaagcggtggagcatgtggtttaattcgaagcaacgcgaagaaccttaccaggccttgacatccccctggatggcccgtaacggggtcagcctttcggggcaggggagacaggtggtgcatggttgtcgtcagctcgtgtcgtgagatgttgggttaagtcccgcaacgagcgcaacccctgcccgcagtagccagcattttagatggggactctgcggggactgccggggacaacccggaggaaggcggggatgacgtcaaatcatcatgccccttatggcctgggctacacacgtgctacaatggcgccgacagagggaggcgaagcggcgacgcggagcgaaccccaaaaacggcgtcccagttcggattgtagtctgcaacccgactacatgaagccggaatcgctagtaatcgcggatcagaatgccgcggtgaatacgttcccgggtcttgtacacaccgcccgtcacaccatgggagccgggaatgcccgaagtctgtgaccgaacccgtaaggggaggggcagccgaaggcaggcccggtgactggggtgaagtcgtaacaaggtagccgt

SEQ ID NO: 30 - DNA, 1489 bp, Clostridium leptum
  rRNA (1)..(1489): 16S rRNA coding gene sequence of Clostridium strain 10
agagtttgatcctggctcaggatgaacgctggcggcgtgcttaacacatgcaagtcgagcgaagcacttttttagaactcttcggagggaagagagggtgacttagcggcggacgggtgagtaacgcgtgggcaacctgccttacacagggggataacaattagaaatgattgctaataccgcataagaccacggtactgcatggtacagtggtaaaaactgaggtggtgtaagatgggcccgcgtctgattaggtagttggtggggtagaagcctaccaagccgacgatcagtagccgacctgagagggcgaccggccacattgggactgagacacggcccaaactcctacgggaggcagcagtggggaatattgcacaatgggggaaaccctgatgcagcgacgccgcgtgagtgaggaagtatttcggtatgtaaagctctatcagcagggaagaaaatgacggtacctgactaagaagcccccggctaactacgtgccagcagccgcggtaatacgtagggggcaagcgttatccggatttactgggtgtaaagggagcgtagacggacttgcaagtctgatgtgaaaatccggggcccaacccgggactgcattgaaactgtattttttggaggggtccgaggaggcaagtggaatcctgggtagcggtgaaatggcgtagaattcagggaggaacaccagtggcggaaggcgaattactggacgataactgacggtgaggcgcgaagcgtgggagcaaacaagaattagataccctggtagtcacgctgtaacgatcgatactaggtgtgcggggactgacccctgcgtgccggagttaacacaataagtatcgcactggggagtacgatcgcaaggttgaaactcaaaggaattgacgggggcccgcacaagcggtggattatgtggtttaattcgaagcaacgcgaagaaccttaccagggcttgacatcctgctaacgaagtagagatacattaggtgcccttcggggaaagcagagacaggtggtgcatggttgtcgtcagctcgtgtcgtgagatgttgggttaagtcccgcaacgagcgcaacccctattgttagttgctacgcaagagcactctagcgagactgccgttgacaaaacggaggaaggcggggacgacgtcaaatcatcatgccccttatgtcctgggctacacacgtaatacaatggcggttaacaaagggatgcaaagccgcgaggcagagcgaaccccaaaaagccgtcccagttcggatcgcaggctgcaacccgcctgcgtgaagtcggaatcgctagtaatcgcggatcagcatgccgcggtgaatacgttcccgggccttgtacacaccgcccgtcacaccatgagagtcgggaacacccgaagtccgtagcctaaccgcaaggagggcgcggccgaaggtgggttcgataattggggtgaagtcgtaacaaggtagccgt

SEQ ID NO: 31 - DNA, 1490 bp, Clostridium leptum
  rRNA (1)..(1490): 16S rRNA coding gene sequence of Clostridium strain 11
agagtttgatcctggctcaggatgaacgctggcggcgtgcttaacacatgcaagtcgaacgagaatccagtgaaggagttttcggacaacggatctggaggaaagtggcggacgggtgagtaacgcgtgagcaatctgccttggagtggggaataacggttggaaacagccgctaataccgcatgatgcgtctgggaggcatctctctggacgccaaagatttatcgctctgagatgagctcgcgtctgattagcttgttggcggggtaaaggcccaccaaggcgacgatcagtagccggactgagaggttggccggccacattgggactgagacacggcccagactcctacgggaggcagcagtggggaatattgggcaatgggcgcaagcctgacccagcaacgccgcgtgaaggaagaaggctttcgggttgtaaacttcttttctgagggacgaagaaagtgacggtacctcaggaataagccacggctaactacgtgccagcagccgcggtaatacgtaggtggcaagcgttatccggatttattgggtgtaaagggcgtgtaggcgggaaagcaagtcagatgtgaaaactcagggctcaaccctgagcctgcatttgaaactgtttttcttgagtgctggagaggcaatcggaattccgtgttgtagcggtgaaatgcgtagattataccggaggaaccaccagtggcggaaggcggattgctggaacagtaactgacgctgaggcgccgaaagcgtggggagcaaacaggatagataccctggtagtccacgccgtaaacgatggatactaagtgtgggggactgaccccttcgtgcccagctaagcaataagtttcccacctggggagtacgatcgcaggtgaaactcaaaggaattgacgggggcccgcccaagcgggtggagtaggggttaattggagcaacgggaagaaccttaccagggcttgacatcctgtaacgaaccagaagagggattaggtgccttcggggaaagcagagacaggtggtgcatggttgtcgtcagctcgtgtcgtgagatgtgggtaaagtcccgcaacgagcgcaacccttattgttagttgctacgcaagagcactctagcgagactgccgttgacaaaacggaggaaggtggggacgacgtcaaatcatcatgccccttacgtcctgggccacacacgtactacaatggcggccaacaaagagaggcaagaccgcgaggtggagaaaatctcaaaaagccgtcccagttcggatcgcaggctgcaacccgcctgcgtgaagttggaatcgctagtaatcgcggatcagcatgccgcggtgaatacgttcccgggccttgtacacaccgcccgtcacaccatgagagtcgggaacacccgaagtccgtagcctaaccgcaaggggggcgcggccgaaggtgggttcgataattggggtgaagtcgtaacaaggtagccgt

SEQ ID NO: 32 - DNA, 1489 bp, Clostridium coccoides
  rRNA (1)..(1489): 16S rRNA coding gene sequence of Clostridium strain 12
agagtttgatcatggctcaggatgaacgctggcggcgtgcttaacacatgcaagtcgaacgggctcatattgaaacctagtgatgtatgagttagtggcggacgggtgagtaacgcgtggagaacctgccgtatactgggggataacacttagaaataggtgctaataccgcataagcgcacagcttcgcatgaagcagtgtgaaaaactccggtggtatacgatggatccgcgtctgattagctggttggcggggtaacagcccaccaaggcgacgatcagtagccggcctgagagggtgaacggccacattgggactgagacacggcccaaactcctacgggaggcagcagtggggaatattgcacaatgggggaaaccctgatgcagcgacgccgcgtgagtgaagaagtatttcggtatgtaaagctctatcagcagggaagaaatactgaccttacggtcagcagacggtacctgactaagaagccccggctaactacgtgccagcagccgcggtaatacgtagggggcaagcgttatccggatttactgggtgtaaagggagcgtagacggcagcgcaagtctgaagtgaaatcccatggcttaaccatggaactgctttggaaactgtgcagctggagtgcaggagaggtaagcggaattcctagtgtagcggtgaatgcgtagatattagaggacaccagtggcgatgcggcttactggactgtactgacgttgagctcgaaagcgtggggagcaccagaattagaatactgtagtcacgccgtaaccgatgatactaggtgtgggggaccaaggtctcgtgccggcggcaaacgcattaagtaatccacctggggagtacgttcgcaagaatgaaactcaaaggaattgacggggacccgcacaagcggtggagcatgtggtttaattcgaagcaacgcgaagaaccttacctggtcttgacatcccgatgacgagtgagcaaagtcactttcccttcggggcattggagacaggtggtgcatggttgtcgtcagctcgtgtcgtgagatgttgggttaagtcccgcaacgagcgcaacccctatttccagtagccagcaggtagagctgggcactctggagagactgcccgggataaccgggaggaaggcggggatgacgtcaaatcatcatgccccttatgatcagggctacacacgtgctacaatggcgtaaacaaagggaagcgagacggtgacgttaagcaaatcccaaaaataacgtcccagttcggattgtagtctgcaactcgactacatgaagctggaatcgctagtaatcgcgaatcagaatgtcgcggtgaatacgttcccgggtcttgtacacaccgcccgtcacaccatgggagtcggaaatgcccgaagtcagtgacctaaccgaaaggaaggagctgccgaaggtggagccggtaactggggtgaagtcgtaacaaggtagccgt

SEQ ID NO: 33 - DNA, 1456 bp, Clostridium coccoides
  rRNA (1)..(1456): 16S rRNA coding gene sequence of Clostridium strain 13
agagtttgatcatggctcaggatgaacgctggcggcgtgcttaacacatgcaagtcgaacgaagcacttgagaacgattcttcggatgaggacttttgtgactgagtggcggacgggtgagtaacgcgtgggtaacctgccctatacagggggataacagttagaaatgactgctaataccgcataagcgcactaaaaccgcatggttcggtgtgaaaaactgaggtggtataggatggacccgcgtctgattagcttgttggtggggtaacggctcaccaaggcgacgatcagtagccggcctgagagggcgaccggccacattgggactgagacacggcccaaactcctacgggaggcagcagtgggggatattgcacaatggggggaaccctgatgcagcgacgccgcgtgggtgaagaagcgcctcggcgcgtaaagccctgtcagcagggaagaaaatgacggtacctgaagaagaagccccggctaactacgtgccagcagccgcggtaatacgtaggggcaagcgttattccgggatttactgggtgtaaagggggcgcagacggcgatgcaagccaggagtgaagcccggggcccacccgggactgctcttggactgcgtgctggagtgcagaaggggcagcgatcctgtgtaccgtgaattgcgtagatatcagagacacgttgcgagcgctgctgactgcactgacgtgagcgaagctggagcacagatagatactgtagtcagcgtaacgatgatactagtgtcgggagcagagactgcccgttgcggcagcccaacgcattagtattccacttggggagtacgtttcgcagaatgaacttcaaggaaatgacggggacccgcacaaggcggtggagcatgtggtttaattcgaagcaacgcgaagaaccttaccaggccttgacatcccccctggatggcccgtaacggggtcagcctttcggggcaggggagacaggtggtgcatggttgtcgtcagctcgtgtcgtgagatgttgggttaagtcccgcaacgagcgcaacccctgcccgcagtagccagcattttagatggggactctgcggggactgccggggacaacccggaggaaggcggggatgacgtcaaatcatcatgccccttatggcctgggctacacacgtgctacaatggcgccgacagagggaggcgaagcggcgacgcggagcgaaccccaaaaacggcgtcccagttcggattgtagtctgcaacccgactacatgaagccggaatcgctagtaatcgcggatcagaatgccgcggtgaatacgttcccgggtcttgtacacaccgcccgtcacaccatgggagccgggaatgcccgaagtctgtgaccgaacccgtaaggggaggggcagccgaaggcaggctcggtgactggggtgaagtcgtaacaaggtagccgt

SEQ ID NO: 34 - DNA, 1475 bp, Clostridium leptum
  rRNA (1)..(1475): 16S rRNA coding gene sequence of Clostridium strain 14
agagtttgatcctggctcaggacgaacgctggcggcgtgcttaacacatgcaagtcgaacggagcacccctgaaggagttttcggacaacggatgggaatgcttagtggcggactggtgagtaacgcgtgaggaacctgccttccagagggggacaacagttggaaacgactgctaataccgcatgatgcgttggagccgcatgactccgacgtcaaagatttatcgctggaagatggcctcgcgtctgattagctagttggtgaggtaacggcccaccaaggcgacgatcagtagccggactgagaggttggccggccacattgggactgagatacggcccagactcctacgggaggcagcagtggggaatattgggcaatggacgcaagtctgacccagcaacgccgcgtgaaggaagaaggctttcgggttgtaaacttcttttaagggggaagagcagaagacggtaccccttgaataagccacggctaactacgtgccagcagccgcggtaatacgtaggtggcaagcgttgtccggatttactgggtgtaaagggcgtgcagccggagagacaagtcagatgtgaaatccacgggctcaacccgtgaactgcatttgaaactgtttcccttgagtgtcggagaggtaatcggaatttccttgtgtagcggtgaatgcgtagatataaggaaggacacagtggcgagcggattactggacgatactgacgtgagcgcgaaagcgtgggggagcaacagaaattagatactgtagtgcagctgtaacgatcgatactagttgcgggactgaccccttgcgtgcgagttacacaataagtatcgcacctgggagtacgatcgcaaggttggaactcaaaggaattgacggggcccgcacaagcgttggattatgtggtttaattcgaagcaacgcgaagaaccttaccagggcttgacatcctgctaacgaagtagagatacattaggtgcccttcggggaaagtagagacaggtggtgcatggttgtcgtcagctcgtgtcgtgagatgttgggttaagtcccgcaacgagcgcaacccctattgttagttgctacgcaagagcactctagcgagactgccgttgacaaaacggaggaaggcggggacgacgtcaaatcatcatgccccttatgtcctgggctacacacgtaatacaatggcggttaacaaagggatgcaaagccgcgaggcagagcgaaccccaaaaagccgtcccagttcggatcgcaggctgcaacccgcctgcgtgaagtcggaatcgctagtaatcgcggatcagcatgccgcggtgaatacgttcccgggccttgtacacaccgcccgtcacaccatgagagtcgggaacacccgaagtccgtagcctaaccgcaaggagggcgcggccgaaggtgggttcgataattggggtgaagtcgtaacaaggtagccgt

SEQ ID NO: 35 - DNA, 1480 bp, Clostridium coccoides
  rRNA (1)..(1480): 16S rRNA coding gene sequence of Clostridium strain 15
agagtttgatcctggctcaggatgaacgctggcggcgtgcttaacacatgcaagtcgaacgggctcatattgaaacctagtgatgtatgagttagtggcggacgggtgagtaacgcgtggagaacctgccgtatactgggggataacacttagaaataggtgctaataccgcataagcgcacagcttcgcatgaagcagtgtgaaaaactccggtggtatacgatggatccgcgtctgattagctggttggcggggtaacagcccaccaaggcgacgatcagtagccggcctgagagggtgaacggccacattgggactgagacacggcccaaactcctacgggaggcagcagtggggaatattgcacaatgggggaaaccctgatgcagcgacgccgcgtgagtgaagaagtatttcggtatgtaaagctctatcagcagggaagaaatactgaccttacggtcagcagacggtacctgactaagaagccccggctaactacgtgccagcagccgcggtaatacgtaggggcaagcgttatccggatttactgggtgtaaagggagcgtagacggcagcgcaagtctgaagtgaaatcccatggcttaacccatggaactgctttggaaactgtgcagctggagtgcaggagaggtaagcggaattcctagtgtagcgtgaaatgcgtagattattaggaggacaacagtgcgagcgctactgacgtgaggctcgaagcgtgggagcaaacaggattagatacctggtagtcacgcgtaaacgatgattactagggtgttgggggaccaaggtcttcggtgccggcgcaaacgcattaagtaatccacctggggagtacgttcgcaagaatgaaactcaaaggaattgacggggacccgcacaagcggtggagcatgtggtttaattcgaagcaacgcgaagaaccttacctggtcttgacatcccgatgacgagtgagcaaagtcactttcccttcggggcattggagacaggtggtgcatggttgtcgtcagctcgtgtcgtgagatgttgggttaagtcccgcaacgagcgcaacccctatttccagtagccagcaggtagagctgggcactctggagagactgcccgggataaccgggaggaaggcggggatgacgtcaaatcatcatgccccttatgatcagggctacacacgtgctacaatggcgtaaacaaagggaagcgagacggtgacgttaagcaaatcccaaaaataacgtcccagttcggattgtagtctgcaactcgactacatgaagctggaatcgctagtaatcgcgaatcagaatgtcgcggtgaatacgttcccgggtcttgtacacaccgcccgtcacaccatgggagtcggaaatgcccgaagtcagtgacctaaccgaaaggaaggagctgccgaaggtggagccggtaactggggtgaagtcgtaacaaggtagccgt

SEQ ID NO: 36 - DNA, 1486 bp, Clostridium papyrosolvens
  rRNA (1)..(1486): 16S rRNA coding gene sequence of Clostridium strain 16
agagtttgatcctggctcaggataaacgctggcggcgcacataagacatgcaagtcgaacggacttaactcattcttttagattgagagcggttagtggcggactggtgagtaacacgtaagcaacctgcctatcagaggggaataacagtgagaaatcattgctaataccgcatatgctcacagtatcacatgatacagtgaggaaaggagcaatccgctgatagatgggcttgcgcctgattagttagttggtggggtaacggcctaccaagacgacgatcagtagccggactgagaggttgaacggccacattgggactgagatacggcccagactcctacgggaggcagcagtcgggaatattgcgcaatggaggaaactctgacgcagtgacgccgcgtataggaagaaggttttcggattgtaaactattgtcgttagggaagataaaagactgtacctaaggaggaagccccggctaactatgtgccagcagccgcggtaatacatagggggcaagcgttatccggaattattgggtgtaaagggtgcgtagacggaagaacaagttggttgtgaaatccctcggctcaactgaggaactgcaaccaaaactattctccttgagtgtcggagaggaaagtggaattcctagtgtagcggtgaaatgcgtagatattaggaggaacaccagtggcgaaggcgactttctggacgataactgacgttgaggcacgaaagtgtggggagcaaacaggattagataccctggtagtccacactgtaaacgatggatactaggtgtagggtgtattaagcactctgtgccgccgctaacgcattaagtatcccacctggggagtacgaccgcaaggttgaaactcaaaggaattgacgggggcccgcacaagcagtggagtatgtggtttaattcgaagcaacgcgaagaaccttaccagggcttgacatataccggaatatactagagatagtatagtccttcgggactggtatacaggtggtgcatggttgtcgtcagctcgtgtcgtgagatgttgggttaagtcccgcaacgagcgcaacccctatcgttagttgctagcaggtaatgctgagaactctagcgagactgccggtgataaatcggaggaaggtggggatgacgtcaaatcatcatgccctttatgtcctgggctacacacgtactacaatggccgtaacagagggaagcaatatagtgatatggagcaaaaccctaaaagcggtctcagttcggattgaaggctgaaattcgccttcatgaagccggaattgctagtaatggcaggtcagcatactgccgtgaatacgttcccgggccttgtacacaccgcccgtcacaccatgagagttggaaatacccgaagcctgtgagctaactgtaaagaggcagcagtcgaaggtagagccaatgattggggtgaagtcgtaacaaggtagccgt

SEQ ID NO: 37 - DNA, 1493 bp, Clostridium leptum
  rRNA (1)..(1493): 16S rRNA coding gene sequence of Clostridium strain 17
agagtttgatcatggctcaggatgaacgctggcggcgtgcttaacacatgcaagtcgaacgagaaccaacggattgaggattcgtccaaatgaagttggggaaagtggcggacgggtgagtaacgcgtgagcaatctgccttggagtggggaataacggttggaaacagccgctaataccgcatgatgcgtctgggaggcatctctctggacgccaaagatttatcgctctgagatgagctcgcgtctgattagctagttggcggggcaacggcccaccaaggcgacgatcagtagccggactgagaggttggccggccacattgggactgagacacggcccagactcctacgggaggcagcagtggggaatattgggcaatgggcgcaagcctgacccagcaacgccgcgtgaaggaagaaggctttcgggttgtaaacttcttttaagggggacgaacaaatgacggtaccccttgaataagccacggctaactacgtgccagcagccgcggtaatacgtaggtggcaagcgttatccggatttattgggtgtaaagggcgtgtaggcgggaatgcaagtcagatgtgaaaactatgggctcaacccatagcctgcatttgaaactgtatttcttgagtgctggagaggcaatcggaattccgtgtgtagcggtgaaatgcgtagatatacggaggaacaccagtggcgaagcggattgctggacagtaactgacgctgaggcgcgaaagcgtggggagcaaacagggattagataccctggtagtcacgccgtaaacgatggatactaggtgtggggggactgaccccctccgtgccgcagctaacgcaataagtatcccacctggggagtacgatcgcaagggttgaaactcaaaggaattgacgggggcccgcacaagcggtggagtatgtggtttaattcgaagcaacgcgaagaaccttaccagggcttgacatcctgctaacgaaccagagatggatcaggtgcccttcggggaaagcagagacaggtggtgcatggttgtcgtcagctcgtgtcgtgagatgttgggttaagtcccgcaacgagcgcaacccctattgttagttgctacgcaagagcactctagcgagactgccgttgacaaaacggaggaaggtggggacgacgtcaaatcatcatgccccttacgtcctgggccacacacgtactacaatggcggccaacaaagagaggcaagaccgcgaggtggagcaaatctcaaaaagccgtcccagttcggatcgcaggctgcaacccgcctgcgtgaagttggaatcgctagtaatcgcggatcagcatgccgcggtgaatacgttcccgggccttgtacacaccgcccgtcacaccatgagagtcgggaacacccgaagtccgtagcctgaccgcaaggggggcgcggccgaaggtgggttcgataattggggtgaagtagtaacaaggtagccgt

SEQ ID NO: 38 - DNA, 1493 bp, Clostridium leptum
  rRNA (1)..(1493): 16S rRNA coding gene sequence of Clostridium strain 18
agagtttgatcctggctcaggacgaacgctggcggcgcgcctaacacatgcaagtcgaacggagcttatatttcagaagttttcggatggacgagagataagcttagtggcggacgggtgagtaacacgtgagcaacctgcctttcagagggggataacagttggaaacgactgctaataccgcataacgctgcgatggggcatcccgatgcagccaaaggagcaatccgctgaaagatgggctcgcggccgattagctagttggtggggcaacggcccaccaaggcgacgatcggtagccggactgagaggttgatcggccacattgggactgagacacggcccagactcctacgggaggcagcagtgggggatattgcacaatggaggaaactctgatgcagcgacgccgcgtgagggaagacggtcttcggattgtaaacctctgtctttggggaagaaaatgacggtacccaaagaggaagctccggctaactacgtgccagcagccgcggtaatacgtacggagcgagcgttgtccggaattactgggtgtaaagggagcgtacgcgggcgagaaagttgaatgttaaatctaccggcttaactggtagctgcgttcaaaacttcttgtcttgagtgaagtagaggcaggcggaattcctagtgtagcggtgaaatgcgtagatataggaggacaccagtgggcgaagccgcctgctgggctttaactgacgctgaggctcgaaagcgtggggagcaaaccaggattagataccctggtagtcaacgctgtaaacgatgattactaggtgtgggggggactgaccccctccgtgccgcagttaacacaataagtatccacctggggagtacggccgcaaagtttgaaaactcaaaaggaatgacgggggcccgcacaaagcagtggagtatgtggtttaatttcgaagcaacgcgaagaaccttaccaggtcttgacatcgtgcgcatagcctagagataggtgaagcccttcggggcgcacagacaggtggtgcatggttgtcgtcagctcgtgtcgtgagatgttgggttaagtcccgcaacgagcgcaacccttattattagttgctacgcaagagcactctaatgagactgccgttgacaaaacggaggaaggtggggatgacgtcaaatcatcatgccccttatgacctgggctacacacgtactacaatggcactgaaacagagggaagcgacatcgcgaggtgaagcgaatcccaaaaaagtgtcccagttcggattgcaggctgcaactcgcctgcatgaagtcggaattgctagtaatcgcggatcagcatgccgcggtgaatacgttcccgggccttgtacacaccgcccgtcacaccatgggagtcggtaacacccgaagccagtagcctaaccgcaaggagggcgctgtcgaaggtgggattgatgactggggtgaagtcgtaacaaggtagccgt

SEQ ID NO: 39 - DNA, 1483 bp, Clostridium leptum
  misc_feature (1)..(1483): 16S rRNA coding gene sequence of Clostridium strain 19
agagtttgatcctggctcaggacgaacgctggcggcacgcctaacacatgcaagtcgaacggagtgaagatgcttgcatctgaacttagtggcggacgggtgagtaacacgtgagcaacctgcctttcagagggggataacgtttggaaacgaacgctaataccgcataaaatatcggagtcgcatggcactgatatcaaaggagcaatccgctgaaagatgggctcgcgtccgattaggcagttggcggggtaacggcccaccaaaccgacaatcggtagccggactgagaggttgaacggccacattgggactgagacacggcccagactcctacgggaggcagcagtgggggatattgcacaatgggggaaaccctgatgcagcgatgccgcgtgaatgaagacggccttcgggttgtaaagttctgtcgcaggggacgaaaatgacggtaccctgcaagaaagctccggctaactacgtgccagcagccgcggtaatacgtagggagcaagcgttgtccggaattactgggtgtaaagggagcgtaggcgggaggataaagttgaatgtgaaatctatgggctcaacccatagctgcgttcaaaactgttcttcttgagtgaagtagaggcaggcggaattcctagtgtagcggtgaaatgcgtagatattaggaggaacaccagtggcgaaagcggcctgctgggcttttactgacgctgaggctcgaaagcgtgggtagcaaacagaattagattaccctgttattcacggcggtaaacgatgattactaggtttgggttgacctgacccccattcgtgccggaagtaacaccataaagtaatccacctgggggagtacggccgccaggttgaaacttcaaaaggaattgacgggggcccgcacaagcagtggaggtatgtggtttaatttcgacgcaaacgcgaagaaccttaccagggtcttgacatcgagtgacggacatagagatatgtctttcctttcgggacacgaagacaggtggtgcatggttgtcgtcagctcgtgtcgtgagatgttgggttaagtcccgcaacgagcgcaacccttaccattagttgctacgcaagagcactctgatgggactgccgttgacaaaacggaggaaggtggggatgacgtcaaatcatcatgccccttatgacctgggcgacacacgtactacaatggcggtcaacagagggaggcaaagccgcgaggcagagcaaacccctaaaagccgtctcagttcggattgcaggctgcaactcgcctgcatgaagtcggaattgctagtaatcgcggatcagcatgccgcggtgaatacgttcccgggccttgtacacaccgcccgtcacaccatgagagccggtaacacccgaagtcaatagtctaaccgcaaggaggacattgccgaaggtgggattggtaattggggtgaagtcgtaacaaggtagccgt

SEQ ID NO: 40 - DNA, 1511 bp, Clostridium coccoides
  rRNA (1)..(1511): 16S rRNA coding gene sequence of Clostridium strain 20
agagtttgatcctggctcaggatgaacgctggcggcgtgcttaacacatgcaagtcgaacgggctcatattgaaacctagtgatgtatgagttagtggcggacgggtgagtaacgcgtggagaacctgccgtatactgggggataacacttagaaataggtgctaataccgcataagcgcacagcttcgcatgaaacagtgtgaaaaactccggtggtatacgatggatccgcgtctgattagctggttggcggggtaacagcccaccaaggcgacgatcagtagccggcctgagagggtgaacggccacattgggactgagacacggcccaaactcctacgggaggcagcagtggggaatattgcacaatgggggaaaccctgatgcagcgacgccgcgtgagtgaagaagtatttcggtatgtaaagctctatcagcagggaagaaatactgaccttacggtcagcagacggtacctgactaagaagccccggctaactacgtgccagcagccgcggtaatacgtaggggcaagcgttatccggatttactgggtgtaaagggagcgtagacggcagcgcaagtctgagtgaaatcccatggcttaaccatggaactgctttggaaactgtgcagctggagtgcaggagaggtaaagcggaattcctagtgtagcgggtgaaatgcgtagatataggaggaacaacagtggcggaaggcggctactgggactgtaactgacgttgaggctcgaaagcgtggggagcaaacaggattagataccctggtagtcacgccgtaaacgatgattactaggtgttgggggaccataggtcttcggtgccggcgcaaacgcaattaagtaatccacctgggggagtacgttcgcaagaatgaaactcaaaggaattgacggggacccgcacaaagcggtggagcatgtggtttaattcgaaagcaaacgcgaagaaaccttacctggtcttgacatcccgatgacgagtgagcaaagtcactttcccttcggggcaattggagacaggtggtgcatgggttgtcgtcagctcgtgtcgtgagatgttgggttaagtcccgcaacgagcgcaacccctatttccagtagccagcaggtagagctgggcactctggagagactgcccgggataaccgggaggaaggcggggatgacgtcaaatcatcatgccccttatgatcagggctacacacgtgctacaatggcgtaaacaaagggaagcgagacggtgacgttaagcaaatcccaaaaataacgtcccagttcggattgtagtctgcaactcgattacatgaagctggaatcgctagtaatcgcgaatcagaatgtcgcggtgaatacgttcccgggtcttgtacacaccgcccgtcacaccatgggagtcggaaatgcccgaagtcagtgacctaaccgaaaggaaggagctgccgaaggtggagccggtaactggggtgaagtagataacaaggtagccgt

SEQ ID NO: 41 - DNA, 1495 bp, Clostridium leptum
  rRNA (1)..(1495): 16S rRNA coding gene sequence of Clostridium strain 21
agagtttgatcctgcgctcaggacgaacgctggcggcgcgcctaacacatgcaagtcgaacgggactattttgggagaagttttcggatggatctcgggatagtttagtggcggacgggtgagtaacgcgtgggcaacctgccttacacagggggataacaattagaaatgattgctaataccgcataagaccacggtactgcatggtacagtggtaaaaactgaggtggtgtaagatgggcccgcgtctgattaggtagttggtggggtagaagcctaccaagccgacgatcagtagccgacctgagagggcgaccggccacattgggactgagacacggcccaaactcctacgggaggcagcagtggggaatattgcacaatgggggaaaccctgatgcagcgacgccgcgtgagtgaggaagtatttcggtatgtaaagctctatcagcagggaagaaaatgacggtacctgactaagaagccccggctaactacgtgccagcagccgcggtaatacgtagggggcaagcgttatccggatttactgggtgtaaagggagcgtagacggacttgcaagtctgatgtgaaaatccgggggcccaaccccggaactgcattggaaactgtatatctagagtgtcggagaggcaagtggaatttcctggtgtagcggtgaaatgcgtagatatcagaggaacaccagtggcgaaggcgcttgcctgacgatgactgacgttgaagctcgaaaagcgtgggtagcaaacagaattagataccctggtaagtcaacccggtaaacgatgattactaggttttggttggactgaccccatccgtgccggagtaacaccaataagttatccaacctgggaagtacggccggcaggttgaaactcaaaaggaaatgacgggggcccgcacaagcagttgaagtatgtgggttaattcgacgcaaacgcgaagaaccttaccaggtcttgacatcgagtgacggacatagagatatgtctttccttcgggacacgaagacaggtggtgcatggttgtcgtcagctcgtgtcgtgagatgttgggttaagtcccgcaacgagcgcaacccttaccattagttgctacgcaagagcactctgatgggactgccgttgacaaaacggaggaaggtggggatgacgtcaaatcatcatgccccttatgacctgggcgacacacgtactacaatggcggtcaacagagggaggcaaagccgcgaggcagagcaaacccctaaaagccgtctcagttcggattgcaggctgcaactcgcctgcatgaagtcggaattgctagtaatcgcggatcagcatgccgcggtgaatacgttcccgggccttgtacacaccgcccgtcacaccatgagagccggtaacacccgaagtcaatagtctaaccgcaaggaggacattgccgaaggtgggattggtaattggggtgaagtcgtaacaaggtagccgt

SEQ ID NO: 42 - DNA, 1491 bp, Clostridium leptum
  rRNA (1)..(1491): 16S rRNA coding gene sequence of Clostridium strain 22
agagtttgatcctggctcaggatgaacgctggcggcgtgcttaacacatgcaagtcgaacgagaatccagtgaaggagttttcggacaacggatctggaggaaagtggcggacgggtgagtaacgcgtgagcaatctgccttggagtggggaataacggttggaaacagccgctaataccgcatgatgcgtctgggaggcatctctctggacgccaaagatttatcgctctgagatgagctcgcgtctgattagcttgttggcggggtaaaggcccaccaaggcgacgatcagtagccggactgagaggttggccggccacattgggactgagacacggcccagactcctacgggaggcagcagtggggaatattgggcaatgggcgcaagcctgacccagcaacgccgcgtgaaggaagaaggctttcgggttgtaaacttcttttctgagggacgaagaaagtgacggtacctcaggaataagccacggctaactacgtgccagcagccgcggtaatacgtaggtggcaagcgttatccggatttattgggtgtaaagggcgtgtaggcgggaaagcaagtcagatgtgaaaactcagggctcaaccctgagcctgcatttgaaactgtttttcttgagtgctggagaggcaatcggaattccgtgtgtagcggtgaaatgcgtagatatacggaggacaccagtggcgaagcggattgctggacagtaactgacgctgaggcgcgaagcgtggggagcaaacaggattagataccctggtagtccacgccgtaaacgatggatactaggtgtggggggactgaccccctccgtgccgcagctaacgcaataagtatcccacctggggagtacgatcgcaaggttgaaactcaaaggaattgacgggggcccgcacaagcggtggagtatgtggtttaattcgaagcaacgcgaagaaccttaccagggcttgacatcctgctaacgaaccagagatggattaggtgcccttcggggaaagcagagacaggtggtgcatggttgtcgtcagctcgtgtcgtgagatgttgggttaagtcccgcaacgagcgcaacccttattgttagttgctacgcaagagcactctagcgagactgccgttgacaaaacggaggaaggtggggacgacgtcaaatcatcatgccccttacgtcctgggccacacacgtactacaatggcggccaacaaagagaggcaagaccgcgaggtggagcaaatctcaaaaagccgtcccagttcggatcgcaggctgcaacccgcctgcgtgaagttggaatcgctagtaatcgcggatcagcatgccgcggtgaatacgttcccgggccttgtacacaccgcccgtcacaccatgagagtcgggaacacccgaagtccgtagcctaaccgcaaggggggcgcggccgaaggtgggttcgataattggggtgaagtcgtaacaaggtagccgt

SEQ ID NO: 43 - DNA, 1495 bp, Clostridium leptum
  rRNA (1)..(1495): 16S rRNA coding gene sequence of Clostridium strain 23
agagtttgatcctgtgcctcaggatgaacgctggcggcgtgcttaacacatgcaagtcgaacgagaaccaacggattgaggattcgtccaaatgaagttggggaaagtggcggacgggtgagtaacgcgtgagcaatctgccttggagtggggaataacggttggaaacagccgctaataccgcatgatgcgtctgggaggcatctctctggacgccaaagatttatcgctctgagatgagctcgcgtctgattagctagttggcggggcaacggcccaccaaggcgacgatcagtagccggactgagaggttggccggccacattgggactgagacacggcccagactcctacgggaggcagcagtggggaatattgggcaatgggcgcaagcctgacccagcaacgccgcgtgaaggaagaaggctttcgggttgtaaacttcttttaagggggacgaacaaatgacggtaccccttgaataagccacggctaactacgtgccagcagccgcggtaatacgtaggtggcaagcgttatccggatttattgggtgtaaagggcgtgtaggcgggaatgcaagtcagatgtgaaaactatgggctcaacccatagcctgcatttgaaactgtatttcttgagtgctggagaggcaatcggaattccgtgtgtagcggtgaaatgcgtagatatacggaggaacaccagtggcgaaggcggattgctggacagtaactgacgctgaggcgcgaaagcgtggggagcaaacaggattagataccctggtagtccacgccgtaaacgatggatactaagtgtggggggactgaccccctccgtgccgcagctaacgcaataagtatcccacctggggagtacgatcgcaaggttgaaactcaaaggaattgacgggggcccgcacaagcggtggagtatgtggtttaattcgaagcaacgcgaagaaccttaccagggcttgacatcctgctaacgaaccagagatggatcaggtgcccttcggggaaagcagagacaggtggtgcatggttgtcgtcagctcgtgtcgtgagatgttgggttaagtcccgcaacgagcgcaacccctattgttagttgctacgcaagagcactctagcgagactgccgttgacaaaacggaggaaggtggggacgacgtcaaatcatcatgccccttacgtcctgggccacacacgtactacaatggcggccaacaaagagaggcaagaccgcgaggtggagcaaatctcaaaaagccgtcccagttcggatcgcaggctgcaacccgcctgcgtgaagttggaatcgctagtaatcgcggatcagcatgccgcggtgaatacgttcccgggccttgtacacaccgcccgtcacaccatgagagtcgggaacacccgaagtccgtagcctgaccgcaaggggggcgcggccgaaggtgggttcgataattggggtgaagtcgtaacaaggtagccgt

SEQ ID NO: 44 - DNA, 1440 bp, Clostridium leptum
  rRNA (1)..(1440): 16S rRNA coding gene sequence of Clostridium strain 24
agagtttgatcctggctcaggacgaacgctggcggcacgcctaacacatgcaagtcgaacggagtgaagatgctcgcatctgaacttagtggcggacgggtgagtaacacgtgagcaacctgcctttcagagggggataacgtttggaaacgaacgctaataccgcataaaatatcggagtcgcatggcactgatatcaaaggagtaatccgctgaaagatgggctcgcgtccgattaggcagttggcggggtaacggcccaccaaaccgacaatcggtagccggactgagaggttgaacggccacattgggactgagacacggcccagactcctacgggaggcagcagtgggggatattgcacaatgggggaaaccctgatgcagcgatgccgcgtgaatgaagacggccttcgggttgtaaagttctgtcgcaggggacgaaaatgacggtaccctgcaagaaagctccggctaactacgtgccagcagccgcggtaatacgtagggagcaagcgttgtccggaattactgggtgtaaagggagcgtaggcgggaggataagttgaatgtgaaatctatgggctcaacccatagttgcgttcaaaactgttcttcttgagtgaagtagaggcaggcggaattcctagtgtagcggtgaaatgcgtagatattagaggaacaccagtggcgaagcggcctgctgggcttttactgacgctgagctcgaaagcgtgggtagcaacaggattagataccctggtagtccacgcggtaaacgatgattactagtgtgggtggactgacccatccatgccggagttaacacaatagtaatccacctggggagtacgcgcagtgaactcaaaggattgacggggcccgcacaagcagtgagtatgtggtttattcgacgcacgcgagactacagtcttgacatcgatgacggactagagatatgtctttctcggacacgaagacaggtggtgcatggttgtcgtcagctcgtgtcgtgagatgttgggttaagtcccgcaacgagcgcaacccttaccattagttgttacgcaagagcactctaatgggactgccgttgacaaaacggaggaaggtggggatgacgtcaaatcatcatgccccttatgacctgggcgacacacgtactacaatggcggtcaacagagggaggcaaagccgcgaggcagagcaaacccctaaaagccgtctcagttcggattgcaggctgcaactcgcctgcatgaagtcggaattgctagtaatcgcggatcagcatgccgcggtgaatacgttcccgggccttgtacacaccgcccgtcacaccatgagagccggtaacacccgaagtcaatagtctaaccgcaaggaggacattgccgaaggtgggatggtaattggggtgaagtagtaacaaggtagccgt

SEQ ID NO: 45 - DNA, 1495 bp, Clostridium leptum
  rRNA (1)..(1495): 16S rRNA coding gene sequence of Clostridium strain 25
agagtttgatcctggctcaggatgaacgctggcggcgtgcttaacacatgcaagtcgaacgagaaccattggatcgaggattcgtccaagtgaaggtggggaaagtggcggacgggtgagtaacgcgtgagcaatctgccttggagtggggaataacggctggaaacagccgctaataccgcatgatacagctgggaggcatctccctggctgtcaaagatttatcgctctgagatgagctcgcgtctgattagctagttggcggggtaacggcccaccaaggcgacgatcagtagccggactgagaggttggccggccacattgggactgagacacggcccagactcctacgggaggcagcagtggggaatattgggcaatgggcgcaagcctgacccagcaacgccgcgtgaaggaagaaggctttcgggttgtaaacttcttttgtcagggacgaagcaagtgacggtacctgacgaataagccacggctaactacgtgccagcagccgcggtaatacgtagtggcaagcgttatccggatttattggggtgtaaagggcgtgtaggcgggaatgcaagtcagatgtgaaaactatggggctcaacccatagcctgcatttgaaactgtatttcttgagtgctggagaggcaatcgaattccgtgtgtagcgggtgaaatgcgtagatatacggaggaacaccagtggcgaagcggattgctggacaagtaactgacgctgaggcgcgaaagcgtggggagcaaacaggattagataccctggtagtccacgccgtaaacgatggatactaggtgtggggggactgaccccctccgtgccgcagctaacgcaataagtatcccacctggggagtacgatcgcaaggttgaaactcaaaggaattgacgggggcccgcacaagcggtggagtatgtggtttaattcgacgcaacgcgaagaaccttaccagggcttgacatcctactaacgaaccagagatggattaggtgcccttcggggaaagtagagacaggtggtgcatggttgtcgtcagctcgtgtcgtgagatgttgggttaagtcccgcaacgagcgcaacccctattgttagttgctacgcaagagcactctagcgagactgccgttgacaaaacggaggaaggtggggacgacgtcaaatcatcatgccccttacgtcctgggccacacacgtactacaatggcggccaacaaagagaggcaaagccgcgaggtggagcaaatctcaaaaagccgtcccagttcggatcgcaggctgcaacccgcctgcgtgaagttggaatcgctagtaatcgcggatcagcatgccgcggtgaatacgttcccgggccttgtacacaccgcccgtcacaccatgagagtcgggaacacccgaagtccgtagcctaaccgcaaggggggcgcggccgaaggtgggttcgataattggggtgaagtcgtaacaaggtagccgt

SEQ ID NO: 46 - DNA, 1495 bp, Clostridium leptum
  rRNA (1)..(1495): 16S rRNA coding gene sequence of Clostridium strain 26
agagtttgatcatggctcaggacgaacgctggcggcgtgcttaacacatgcaagtcgaacggagcacccctgaaggagttttcggacaacggatgggaatgcttagtggcggactggtgagtaacgcgtgaggaacctgccttccagagggggacaacagttggaaacgactgctaataccgcatgatgcgttggagccgcatgactccgacgtcaaagatttatcgctggaagatggcctcgcgtctgattagctagttggtgaggtaacggcccaccaaggcgacgatcagtagccggactgagaggttggccggccacattgggactgagatacggcccagactcctacgggaggcagcagtggggaatattgggcaatggacgcaagtctgacccagcaacgccgcgtgaaggaagaaggctttcgggttgtaaacttcttttaagggggaagagcagaagacggtaccccttgaataagccacggctaactacgtgccagcagccgcggtaatacgtaggtggcaagcgttgtccggatttactgggtgtaaagggcgtgcagccggagagacaagtcagatgtgaaatccacgggctcaacccgtgaactgcatttgaaactgtttcccttgagtgtcggagagggtaatcggaattcctttgtgtagcggtgaaatgcgtagatataagaagaacaccagtggcgaaggcggattactggacgataactgacggtgaggcgcgaaagcgtgggggagcaacagattaaataccctggtagtccacgctgttaacgatcgatactaggtgtgccgggactgaccccctgcgtgcccggagttaaccacaataagtatcgcacctggggagtacgatcgcaaggtgaacttcaaaggaattgacgggggcccgccccaagccgtggattatgtggttaattcgaagcaacgcgaagaacctacccagggcttgacatcctgctaacgaagtagagatacattaggtgccctttcggggaaagcagagacaggtggtgcatggttgtcgtcagctcgtgtcgtgagatgttgggttaagtcccgcaacgagcgcaacccctattgttagttgctacgcaagagcactctagcgagactgccgttgacaaaacggaggaaggcggggacgacgtcaaatcatcatgccccttatgtcctgggctacacacgtaatacaatggcggttaacaaagggatgcaaagccgcgaggcagagcgaaccccaaaaagccgtcccagttcggatcgcaggctgcaacccgcctgcgtgaagtcggaatcgctagtaatcgcggatcagcatgccgcggtgaatacgttcccgggccttgtacacaccgcccgtcacaccatgagagtcgggaacacccgaagtccgtagcctaaccgcaaggagggcgcggccgaaggtgggttcgataattggggtgaagtcgtaacaaggtagccgt

SEQ ID NO: 47 - DNA, 1509 bp, Clostridium leptum
  rRNA (1)..(1509): 16S rRNA coding gene sequence of Clostridium strain 27
agagtttgatcctggctcaggatgaacgctggcggcgtgcttaacacatgcaagtcgaacggagtacccctgaaggagttttcggacaactgatgggactacttagtggcggacgggtgagtaacgcgtgagtaacctgccttggagtggggaataacagctggaaacagctgctaataccgcataatatgtctgtgtcgcatggcactggacatcaaagatttatcgctctgagatggactcgcgtctgattagctagttggcggggtaacggcccaccaaggcgacgatcagtagccggactgagaggttggccggccacattgggactgagacacggcccagactcctacgggaggcagcagtggggaatattgggcaatgggcgcaagcctgacccagcaacgccgcgtgaaggaagaaggctttcgggttgtaaacttcttttaagggggaagagcagaagacggtaccccttgaataagccacggctaactacgtgccagcagccgcggtaatacgtaggtggcaagcgttgtccggatttactgggtgtaaagggcgtgcagccggagagacaagtcagatgtgaaatccacgggctcaacccgtgaactgcatttgaaactgtttcctggagttcggagggtatggaattcttgttagcggtgaaatgctgtagatatgggagaaccaccagtgcgagggggcttccgggactgtacttgactgtagaggtctcaaagctgggggagcaccgaggaatgagataccgtgatagtcccacgcggtaacggatgattactaggtgttggggggacccaggctctttcggtgccgggcgcaaaccctttaggaattccacctggggaattacgtttggcaagaaaggaacttcaaagaaattgaacgggggacccccccaaccggtggaggcatggtgttttatttcggaggaacgggaagaacctttaccttgttctgaccttccggatgacgaagtgagcaaagtcaacttcccttcggggccatggaggacaggtggtggcatggttggtcgtcagctcgtgtcgtgagatgttgggttaagtcccgcaacgagcgcaacccctatttccagtagccagcaggtagagctgggcactctggagagactgcccgggataaccgggaggaaggcggggatgacgtcaaatcatcatgccccttatgatcagggctacacacgtgctacaatggcgtaaacaaagggaagcgagacggtgacgttaagcaaatcccaaaaataacgtcccagttcggattgtagtctgcaactcgactacatgaagctggaatcgctagtaatcgcgaatcagaatgtcgcggtgaatacgttcccgggtcttgtacacaccgcccgtcacaccatgggagtcggaaatgcccgaagtcagtgacctaaccgaaaggaaggagctgccgaaggtggagccggtaactggggtgaagtcgtaacaaggtagccgt

SEQ ID NO: 48 - DNA, 1583 bp, Clostridium leptum
  rRNA (1)..(1583): 16S rRNA coding gene sequence of Clostridium strain 28
agagtttgatcctggctcaggacgaacgctggcggcgcgcctaacacatgcaagtcgaacggagcttatatttcagaagttttcggatggacgagagataagcttagtggcggacgggtgagtaacacgtgagcaacctgcctttcagagggggataacagttggaaacgactgctaataccgcataacgctgcgatggggcatcccgatgcagccaaaggagcaatccgctgaaagatgggctcgcggccgattagctagttggtggggcaacggcccaccaaggcgacgatcggtagccggactgagaggttgatcggccacattgggactgagacacggcccagactcctacgggaggcagcagtgggggatattgcacaatggaggaaactctgatgcagcgacgccgcgtgagggaagacggtcttcggattgtaaacctctgtctttggggaagaaaatgacggtacccaaagaggaagctccggctaactacgtgccagcagccgcggtaatacgtaggggagcgagcgttgtccggaattactgggtgtaaagggagcgtagcgggcgagaaagttgaatgttaaatctaccggcttaactggtagctgcgtccaaaacttcttggtcttgagtgaaagtaagaggccagggcggaaattcttagtgtaagcgggtgaaaatgcgttagatattagggaggaaccaccaggtgggcgaagggcggcttgctgggctttaactggacggctggaggcttggaaaaggcgtggggagagcaaacacagggaattaagtataccctggtatatgtcacacgcttgtaaagagtatgattaacttagggtggtggggggaacttgaccctttcgtgtgcgcgcaggttaacacacatttagagtatatccaacttggggagagtacggccggcaaagtttgaaacttcaaaagggaaattgagaccggggggcccggccaccaagcacagtggagagtatggtgggtttaatttcgagaagcaaccggcggaagagaaactttaccagtccttgacatcggtggcggcataagccctagagattaggtgaagcccttcgggggccccaccagacaggtggtgcatggttgtcgtcagctcgtgtcgtgagatgttgggttaagtccccgcaaacgagcgcaacccttattattagtttgctacgcaagagcactctaatgagactgccgttgacaaaacggaggaaggtggggatgacgtcaaatcatcatgccccttatgacctgggctacacacgtactacaatggcactgaaacagagggaagcgacatcgcgaggtgaagcgaatcccaaaaaagtgtcccagttcggattgcaggctgcaactcgcctgcatgaagtcggaattgctagtaatcgcggatcagcatgccgcggtgaatacgttcccgggccttgtacacaccgcccgtcacaccatgggagtcggtaacacccgaagccagtagcctaaccgcaaggagggcgctgtcgaaggtgggattgatgactggggtgaagtcgtaacaaggtagccgt

SEQ ID NO: 49 - DNA, 1519 bp, Clostridium coccoides
  rRNA (1)..(1519): 16S rRNA coding gene sequence of Clostridium strain 29
agagtttgatcatggctcaggatgaacgctggcggcgtgcctaacacatgcaagtcgaacgggtgtacgggaaggaaggcttcggccggaaaacctgtgcatgagtggcggacgggtgagtaacgcgtgggcaacctggcctgtacagggggataacacttagaaataggtgctaataccgcataacgggggaagccgcatggcttttccctgaaaactccggtggtacaggatgggcccgcgtctgattagccagttggcagggtaacggcctaccaaagcgacgatcagtagccggcctgagagggcggacggccacactgggactgagacacggcccagactcctacgggaggcagcagtgggggatattgcacaatggggggaaccctgatgcagcgacgccgcgtgggtgaagaagcgcctcggcgcgtaaagccctgtcagcagggaaagaaaatgacggtacctgaagaagaagccccgggctaactacgtgccagcagccggcggtaattacgtaggggggcaggcgttatccggatttactgggtggtaaaggggggcgcaaacggcgatggcaggccaggaatggaaagcccgggggcccaaccccgggacttgctcttgggaaactggcttggctgggagtggcaggaggggcaggcggaaattcctggtggtagcggtggaaaatggctaaaaatcaagaagaaaaaccggtggggaaaggcggcctggtgggactgcgaactgacgttgaaggcccgaaagcgtggggaacaaacaggatagattccctggtagttccacgccgtaaacgatgattactaggtgtcggggagcagagactgcccggtgccgcagccaacgcattaagtaatccacctggggagtacgttcgcaagaatgaaactcaaaggaattgacggggacccgcacaagcggtggagcatgtggtttaattcgaagcaacgcgaagaaccttacctggtcttgacatcccgatgacgagtgagcaaagtcactttcccttcggggcattggagacaggtggtgcatggttgtcgtcagctcgtgtcgtgagatgttgggttaagtcccgcaacgagcgcaacccctatttccagtagccagcaggtagagctgggcactctggagagactgcccgggataaccgggaggaaggcggggatgacgtcaaatcatcatgccccttatgatcagggctacacacgtgctacaatggcgtaaacaaagggaagcgagacggtgacgttaagcaaatcccaaaaataacgtcccagttcggattgtagtctgcaactcgactacatgaagctggaatcgctagtaatcgcgaatcagaatgtcgcggtgaatacgttcccgggtcttgtacacaccgcccgtcacaccatgggagtcggaaatgcccgaagtcagtgacctaaccgaaaggaaggagctgccgaaggtggagccggtaactggggtgaagtcgtaacaaggtagccgt

SEQ ID NO: 50 - DNA, 1497 bp, Clostridium coccoides
  rRNA (1)..(1497): 16S rRNA coding gene sequence of Clostridium strain 30
agagtttgatcctggctcaggatgaacgctggcggcgtgcctaacacatgcaagtcgaacggggtatataagcggaagtttacggatggaaggttatatacttagtggcggacgggtgagtaacgcgtgggcaacctgccccgtgccgggggataccgcctggaaacaggcgctaataccgcataagcgcatacagccgcatgggtgtatgcggaaagctccggcggcacgggatgggcccgcgcccgattagccagttggcggggtaacggcccaccaaagcgacgatcggtagccggcctgagagggcggacggccacattgggactgagacacggcccaaactcctacgggaggcagcagtggggaatattgcacaatgggggaaaccctgatgcagcaacgccgcgtgggtgaaggagcgtttcggcgcgtaaagccctgtcagcggggaagaagaaagacggtacccgaccaagaagccccggctaactacgtgccagcagccgcggtaatacgtagggggcgagcgttatccggaattactgggtgtaaagggagcgtagacggcgaggtaagcctgaagtggaagcccgcggcccaaccgcggaactgctttgggaactgttttgctggagtatgggaggggtaagcggaattcctggtgtagcggtgaaatgcgtagatatcaggaggaacaccggtggcgaaggcggcttactggaccataactgacgttgaggctcgaaagcgtggggagcgaacaggattagataccctggtagtccacgcgtaaacgatgattaccaggtgtcgggtgtcgaaggacggcccggtgccgcagcgaacgcagtaagtaatccacctggggagtacgttcgcaagaatgaaactcaaaggaattgacggggacccgcacaagcggtggagcatgtggtttaattcgaagcaacgcgaagaaccttacccggccttgacatcccctggacagcatatgtaatgtatgtttccttcgggaccagggagacaggtggtgcatggttgtcgtcagctcgtgtcgtgagatgttgggtcaagtcccgcaacgagcgcaacccctgcccccagtagccagcatttaagatgggcactctggggggactgccggggataacccggaggaaggcggggatgacgtcaaatcatcatgccccttatggccggggctacacacgtgctacaatggcgtaaacagagggaggcgagacagcgatgttaagcgaaccccaaaaataacgtcccagttcggattgcagcctgcaactcggctgcatgaagctggaatcgctagtaatcgcggatcagaatgccgcggtgaatacgttcccgggtcttgtacacaccgcccgtcacaccatgggagtcgggaacgcccgaagccggtgaccgaacccgaaaggggaggagccgtcgaaggcgggcctggtgactggggtgaagtcgtaacaaggtagccgt

SEQ ID NO: 51 - DNA, 1475 bp, Clostridium leptum
  rRNA (1)..(1475): 16S rRNA coding gene sequence of Clostridium strain 31
gagtttgatcctggctcaggataaacgctggcggcgcacataagacatgcaagtcgaacgaacttaataccttgcttgcaaggtaagcggttagtggcggactggtgagtaacacgtaagaaatctgcctatcagaggggaataacagtgagaaatcactgctaataccgcatatgccatagttatcgcatgataatagtgggaaagaagcaattcgctgatagatgagcttgcggctgattagctagttggtggggtaacggcctaccaaggcgacgatcagtagccggcctgagagggtgaacggccacattgggactgagacacggcccaaactcctacgggaggcagcagtggggaatattgcacaatgggggaaaccctgatgcagcgacgccgcgtgagtgaagaagtatttcggtatgtaaagctctatcagcagggaagaaaatgacggtacctgactaagaaagccccggctaactacgtgccagcagccgcggtaatacgtagggggcaagcgttatccggatttactggtgtaaagggagcgtagacggcagcgcaagtctgagtgaaatcccatggcttacccatgaaactgctttggaaactgtgcagctggagtgcaggagaggtaagcggaatcctagtgtagcggttgaaatgcgtagattatcagaaggaacaccggtggccgaggcggcctgctgggcttttactgacgctgaggctcgaagcgtgggtagcaaacaggattagataccctggtagtccacgcggtaaacgatgattactaggtgtgggtggactgaccccatccgtgccggagttaacacaataagtaatccacctggggagtacggccgcaaggttgaaactcaaaggaattgacgggggcccgcacaagcagtggagtatgtggtttaattcgacgcaacgcgaagaaccttaccaggtcttgacatcgagtgacggacatagagatatgtctttccttcgggacacgaagacaggtggtgcatggttgtcgtcagctcgtgtcgtgagatgttgggttaagtcccgcaacgagcgcaacccttaccattagttgctacgcaagagcactctaatgggactgccgttgacaaaacggaggaaggtggggatgacgtcaaatcatcatgccccttatgacctgggcgacacacgtactacaatggcggtcaacagagggaggcaaagccgcgaggcagagcaaacccctaaaagccgtctcagttcggattgcaggctgcaactcgcctgcatgaagtcggaattgctagtaatcgcggatcagcatgccgcggtgaatacgttcccgggccttgtacacaccgcccgtcacaccatgagagccggtaacacccgaagtcaatagtctaaccgcaaggaggacattgccgaaggtgggattggtaattggggtgaagtcgtaacaaggtagccgt

SEQ ID NO: 52 - DNA, 1491 bp, Clostridium leptum
  rRNA (1)..(1491): 16S rRNA coding gene sequence of Clostridium strain 32
agagtttgatcctggctcaggatgaacgctggcggcgtgcttaacacatgcaagtcgaacgagaatcagtggattgaggattcgtccaaatgaaactgaggaaagtggcggacgggtgagtaacgcgtgagcaatctgccttggagtggggaataacggctggaaacagccgctaataccgcatgatacagttgggaggcatctctctgactgtcaaagatttatcgctctgagatgagctcgcgtctgattagctagttggcggggtaacggcccaccaaggcgacgatcagtagccggactgagaggttggccggccacattgggactgagacacggcccagactcctacgggaggcagcagtggggaatattgggcaatgggcgcaagcctgacccagcaacgccgcgtgaaggaagaaggctttcgggttgtaaacttcttttctgggggacgaacaaatgacggtaccccaggaataagccacggctaactacgtgccagcagccgcggtaatacgtaggtggcaagcgttatccggatttattgggtgtaaagggcgtgtaggcgggaatgcaagtcagatgtgaaaactatgggctcaacccatagcctgcatttgaaactgtatttcttgagtgctggagaggcaatcggaattccgtgtgtagcggtgaaatgcgtagatatacggaggaacaccagtggcgaagcggattgctggacagtaactgacgctgaggcgcgaaagcgtggggagcaaacaggattagataccctggtagtccacgccgtaacgatggatactagtgtggggggactgaccccctccgtgccgcagctaacgcaataagtatccccacctggggagtacgatcgcaaggttgaaactcaaaggaattgacgggggcccgcacaagcggtggagtatgtggtttaattcgaagcaacgcgaagaaccttaccagggcttgacatcctgctaacgaaccagagatggattaggtgcccttcggggaaagcagagacaggtggtgcatggttgtcgtcagctcgtgtcgtgagatgttgggttaagtcccgcaacgagcgcaacccctattgttagttgctacgcaagagcactctagcgagactgccgttgacaaaacggaggaaggtggggacgacgtcaaatcatcatgccccttacgtcctgggccacacacgtactacaatggcggttaacaaagagaggcaagaccgcgaggtggagcaaatctcaaaaagccgtcccagttcggatcgcaggctgcaacccgcctgcgtgaagttggaatcgctagtaatcgcggatcagcatgccgcggtgaatacgttcccgggccttgtacacaccgcccgtcacaccatgagagtcgggaacacccgaagtccgtagcctaaccgcaaggggggcgcggccgaaggtgggttcgataattggggtgaagtcgtaacaaggtagccgt

SEQ ID NO: 53 - DNA, 1495 bp, Clostridium coccoides
  rRNA (1)..(1495): 16S rRNA coding gene sequence of Clostridium strain 33
agagtttgatcctggctcaggatgaacgctggcggcgtgcctaacacatgcaagtcgaacgggtgtacggggaggaaggcttcggccggaaaacctgtgcatgagtggcggacgggtgagtaacgcgtgggcaacctggcctgtacagggggataacacttagaaataggtgctaataccgcataacgggggaagccgcatggcttttccctgaaaactccggtggtacaggatgggcccgcgtctgattagccagttggcagggtaacggcctaccaaagcgacgatcagtagccggcctgagagggcggacggccacactgggactgagacacggcccagactcctacgggaggcagcagtgggggatattgcacaatggggggaaccctgatgcagcgacgccgcgtgggtgaagaagcgcctcggcgcgtaaagccctgtcagcagggaagaaaatgacggtacctgaagaagaagccccggctaactacgtgccagcagccgcggtaatacgtagggggcaagcgttatccggatttactgggtgtaaagggggcgcagacggcgatgcaagccaggagtgaaagcccggggcccaaccccgggactgctcttggaactgcgtggctggagtgcaggaggggcaggcggaattcctggtgtagcggtgaaatgcgtagatatcagaggaacaccggtggcgaaagcggcctgctggactgcaactgacgttgaggcccgaaagcggtgggagcaaacaggattagataccctggtagtccacgccgtaaacgatgattactaggtgtcggggagcagagactgcccggtgccgcagcccaacgcattaagtatccacctggggagtacgttcgcaagaatgaaactcaaaggaattgacggggacccgcacaagcggtggagcatgtggtttaattcgaagcaacgcgaagaaccttaccaggccttgacatccccctggatggcccgtaacggggccagccctttttgggcaggggagacaggtggtgcatggttgtcgtcagctcgtgtcgtgagatgttgggttaagtcccgcaacgagcgcaacccctgcccgcagtagccagcattttagatggggactctgcggggactgccggggacaacccggaggaaggcggggatgacgtcaaatcatcatgccccttatggcctgggctacacacgtgctacaatggcgccgacagagggaggagaagcggcgacgcggagcgaaccccaaaaacggcgtcccagttcggattgtagtctgcaacccgactacatgaagccggaatcgctagtaatcgcggatcagaatgccgcggtgaatacgttcccgggtcttgtacacaccgcccgtcacaccatgggagccgggaatgcccgaagtctgtgaccgaacccgtaaggggaggggcagccgaaggcaggcccggtgactggggtgaagtcgtaacaaggtagccgt

SEQ ID NO: 54 - DNA, 1493 bp, Clostridium leptum
  rRNA (1)..(1493): 16S rRNA coding gene sequence of Clostridium strain 34
agagtttgatcctggctcaggacgaacgctggcggcgtgcttaacacatgcaagtcgaacggagcacccctgaaggagttttcggacaacggatgggaatgcttagtgtcggactggtgagtaacgcgtgaggaacctgccttccagagggggacaacagttggaaacgactgctaataccgcatgatgcgttggagccgcatgactccgacgtcaaagatttatcgctggaagatggcctcgcgtctgatttgttagttggtgaggtaacggcccaccaaggcgacgatcagtagccggactgagaggttggccggccacattgggactgagatacggcccagactcctacgggaggcagcagtggggaatattgggcaatggacgcaagtctgacccagcaacgccgcgtgaaggaagaaggctttcgggttgtaaacttcttttaagggggaagagcagaagacggtaccccttgaataagccacggctaactacgtgccagcagccgcggtaatacgtaggtggcaagcgttgtccggatttactgggtgtaaagggcgtgcagccggagagacaagtcagatgtgaaatccacgggctcaacccgtgaactgcatttgaaactgtttcccttgagtgtcggagaggtaatcggaattccttgtgtagcggtgaaatgcgtagatataaggaagaacaccagtggcgaaggcggattactggacgataactgacggtgaggcgcgaaagcgtggggagcaaacaggattagataccctggtagtccacgctgtaaacgatcgatactaggtgtgcggggactgaccccctgcgtgccggagttaacacaataagtatcgcacctggggagtacgatcgcaaggttgaaactcaaaggaattgacgggggcccgcacaagcggtggattatgtggtttaattcgaagcaacgcgaagaaccttaccagggcttgacatcctgctaacgaagtagagatacattaggtgcccttcggggaaagcagagacaggtggtgcatggttgtcgtcagctcgtgtcgtgagatgttgggttaagtcccgcaacgagcgcaacccctattgttagttgctacgcaagagcactctagcgagactgccgttgacaaaacggaggaaggcggggacgacgtcaaatcatcatgccccttatgtcctgggctacacacgtaatacaatggcggttaacaaagggatgcaaagccgcgaggcagagcgaaccccaaaaagccgtcccagttcggatcgcaggctgcaacccgcctgcgtgaagtcggaatcgctagtaatcgcggatcagcatgccgcggtgaatacgttcccgggccttgtacacaccgcccgtcacaccatgagagtcgggaacacccgaagtccgtagcctaaccgcaaggagggcgcggccgaaggtgggttcgataattggggtgaagtcgtaacaaggtagccgt

SEQ ID NO: 55 - DNA, 1498 bp, Clostridium coccoides
  rRNA (1)..(1498): 16S rRNA coding gene sequence of Clostridium strain 35
agagtttgatcctggctcaggatgaacgctggcggcgtgcctaacacatgcaagtcgaacgggtgtacagaagggaagattacggtcggaaggtctgtgcatgagtggcggacgggtgagtaacgcgtgggcaacctggcctgtacagggggataacacttagaaataggtgctaataccgcataacgggggaagccgcatggcttttccctgaaaactccggtggtacaggatgggcccgcgtctgattattttttttgtcagggtaacggcctaccaaagcgacgatcagtagccggcctgagagggcggacggccacactgggactgagacacggcccagactcctacgggaggcagcagtgggggatattgcacaatggggggaaccctgatgcagcgacgccgcgtgggtgaagaagcgcctcggcgcgtaaagccctgtcagcagggaagaaaatgacggtacctgaagaagaagccccggctaactacgtgccagcagccgcggtaatacgtaaggggcaagcgttatccggatttactgggtgtaaagggggcgcagacggcgatgcaagccaggagtgaaagcccggggcccaaccccgggactgctcttgggaactgcggtggctggagtgcaggaggggcaggccggaattcctggtgtagcggtgaaatgcgtagatatcaggaggaacaccggtggcgaaggcggcctgctggactgcaactgacgttgaggcccgaaagcgtggggagcaaacaggattagataccctggtagtcacgccgtaaacgatgattactaggtgtcggggagcagagactgcccggtgccgcagccaacgcattaagtaatccacctggggagtacgttcgcaagaatgaaactcaaaggaattgacggggacccgcacaagcggtggagcatgtggtttaattcgaagcaacgcgaagaaccttaccaggccttgacatccccctggatggcccgtaacggggtcagcctttcggggcaggggagacaggtggtgcatggttgtcgtcagctcgtgtcgtgagatgttgggttaagtcccgcaacgagcgcaacccctgcccgcagtagccagcattttagatggggactctgcggggactgccggggacaacccggaggaaggcggggatgacgtcaaatcatcatgccccttatggcctgggctacacacgtgctacaatggcgccgacagagggaggcgaagcggcgacgcggagcgaaccccaaaaacggcgtcccagttcggattgtagtctgcaacccgactacatgaagccggaatcgctagtaatcgcggatcagaatgccgcggtgaatacgttcccgggtcttgtacacaccgcccgtcacaccatgggagccgggaatgcccgaagtctgtgaccgaacccgtaaggggaggggcagccgaaggcaggcccggtgactggggtgaagtcgtaacaaggtagccgt

SEQ ID NO: 56 - DNA, 1491 bp, Clostridium leptum
  rRNA (1)..(1491): 16S rRNA coding gene sequence of Clostridium strain 36
agagtttgatcatggctcaggacgaacgctggcggcaagcttaacacatgcaagtcgaacggagcgcctatgaaggagatttcggtcaacggaataggctgcttagtggctgacgggtgagtaacgcgtgaggaacctgcctttcagagggggacaacagttggaaacgactgctaataccgcataacacataggtgtcgcatggcatttatgtcaaagatttatcgctgaaagatggcctcgcgtctgattagctagttggtgaggtaacggctcaccaaggcgacgatcagtagccggactgagaggttagccggccacattgggactgagatacggcccagactcctacgggaggcagcagtggggaatattgggcaatggacgcaagtctgacccagcaacgccgcgtgaaggaagaaggctttcgggttgtaaacttcttttaagagggaagagcagaagacggtacctcttgaataagccacggctaactacgtgccagcagccgcggtaatacgtagtggcaagcgttgtccggatttactgggtgtaaagggcgtgtagccgggctgacagtcagatgtgaaattccggggctcaaccccggacctgcatttgaaactgttggtcttgagtatcggagaggcaggcggaattcctagtgtagcggtgaaatgcgtagatattaggaggaacaccagtggcgaaggcggcctgctggacgacaactgacggtgaggcgcgaaagcgtggggagcaaacaggattagataccctggtagtccacgctgtaaacgatggatactaggtgtgcggggactgaccccctgcgtgccgcagttaacacaataagtatcccacctggggagtacgatcgcaaggttgaaactcaaaggaattgacgggggcccgcacaagcggtggattatgtggtttaattcgatgcaacgcgaagaaccttaccagggcttgacatcctgctaacgaggtagagatacgtcaggtgcccttcggggaaagcagagacaggtggtgcatggttgtcgtcagctcgtgtcgtgagatgttgggttaagtcccgcaacgagcgcaacccttattgttagttgctacgcaagagcactctagcgagactgccgttgacaaaacggaggaaggtggggacgacgtcaaatcatcatgccccttatgtcctgggctacacacgtaatacaatggcggtaaacagagggatgcaatactgcgaagtggagcgaacccctaaaagccgtcccagttcagattgcagtctgcaactcgactgcatgaagtcggaatcgctagtaatcgcggatcagcatgccgcggtgaatacgttcccgggccttgtacacaccgcccgtcacaccatgagagtcgggaacacccgaagtccgtagcctaaccgcaaggagggcgcggccgaaggtgggttcgataattggggtgaagtcgtaacaaggtagccgt

SEQ ID NO: 57 - DNA, 1493 bp, Clostridium coccoides
  rRNA (1)..(1493): 16S rRNA coding gene sequence of Clostridium strain 37
agagtttgatcctggctcaggatgaacgctggcggcgtgcctaacacatgcaagtcgaacgggtgtacggggaggaaggcttcggccggaaaacctgtgcatgagtggcggacgggtgagtaacgcgtgggcaacctggcctgtacagggggataacacttagaaataggtgctaataccgcataacgggggaagccgcatggcttttccctgaaaactccggtggtacaggatgggcccgcgtctgattagccagttggcagggtaacggcctaccaaagcgacgatcagtagccggcctgagagggcggacggccacactgggactgagacacggcccagactcctacgggaggcagcagtgggggatattgcacaatggggggaaaccctgatgcagcgacgccgcgtgagtgaagaagtatttcggtatgtaaagctctatcagcagggaagaaaatgacggtacctgactaagaagccccggctaactacgtgccagcagccgcggtaatacgtagggggcaagcgttatccggatttactgggtgtaaagggagcgtagacggcagcgcaagtctgaagtgaaatcccatggcttaaccatggaactgctttggaaactgtgcagctggagtgcaggagaggtaagcggaattcctagtgtagcggtgaaatgcgtagatattaggaggaacaccagtggcgaaggcggcttactggactgtactgacgttgaggctcgaaagcgtggggagcaaacaggattagataccctggtagtccacgccgtaaacgatgattactaggtgttgggggaccaaggtcttcggtgccggcgcaaacgcattaagtaatccacctggggagtacgttcgcaagaatgaaactcaaaggaattgacggggacccgcacaagcggtggagcatgtggtttaattcgaagcaacgcgaagaaccttacctggtcttgacatcccgatgacgagtgagcaaagtcactttcccttcggggcattggagacaggtggtgcatggttgtcgtcagctcgtgtcgtgagatgttgggttaagtcccgcaacgagcgcaacccctatttccagtagccagcaggtagagctgggcactctggagagactgcccgggataaccgggaggaaggcggggatgacgtcaaatcatcatgccccttatgatcagggctacacacgtgctacaatggcgtaaacaaagggaagcgagacggtgacgttgagcaaatcccaaaaataacgtcccagttcggattgtagtctgcaactcgactacatgaagctggaatcgctagtaatcgcgaatcagaatgtcgcggtgaatacgttcccgggtcttgtacacaccgcccgtcacaccatgggagtcggaaatgcccgaagtcagtgacctaaccgaaaggaaggagctgccgaaggtggagccggtaactggggtgaagtcgtaacaaggtagccgt

SEQ ID NO: 58 - DNA, 1493 bp, Clostridium leptum
  rRNA (1)..(1493): 16S rRNA coding gene sequence of Clostridium strain 38
aaagtttgatcctggctcaggacgaacgctggcggcgtgcttaacacatgcaagtcgaacggagcacccctgaaggagttttcggacaacggatgggaatgcttagtggcggactggtgagtaacgcgtgaggaacctgccttccagagggggacaacagttggaaacgactgctaataccgcatgatgcgttggagccgcatgactccgacgtcaaagatttatcgctggaagatggcctcgcgtctgattagctagttggtgaggtaacggcccaccaaggcgacgatcagtagccggactgagaggttggccggccacattgggactgagatacggcccagactcctacgggaggcagcagtggggaatattgggcaatggacgcaagtctgacccagcaacgccgcgtgaaggaagaaggctttcgggttgtaaacttcttttaagggggaagagcagaagacggtaccccttgaataagccacggctaactacgtgccagcagccgcggtaatacgtagtggcaagcgttgtccggatttactgggtgtaaagggcgtgcagccggagagacaagtcagatgtgaaatccacgggctcaacccgtgaactgcatttgaaactgtttcccttgagtgtcggagaggtaatcggaattccttgtgtagcggtgaaatgcgtagatataaggaagaacaccagtggcgaaggcggattactggacgataaactgacggtgaggcgcgaaagcgtggggagcaaacaggattagataccctggtagtccacgctgtaaacgatcgatactaggtgtgcggggactgaccccctgcgtgccggagttaacacaataagtatcgcacctggggagtacgatcgcaaggttgaaactcaaaggaattgacgggggcccgcacaagcggtggattatgtggtttaattcgaagcaacgcgaagaaccttaccagggcttgacatcctgctaacgaagtagagatacattaggtgcccttcggggaaagtagagacaggtggtgcatggttgtcgtcagctcgtgtcgtgagatgttgggttaagtcccgcaacgagcgcaacccctattgttagttgctacgcaagagcactctagcgagactgccgttgacaaaacggaggaaggcggggacgacgtcaaatcatcatgccccttatgtcctgggctacacacgtaatacaatggcggttaacaaagggatgcaaagccgcgaggcagagcgaaccccaaaaagccgtcccagttcggatcgcaggctgcaacccgcctgcgtgaagtcggaatcgctagtaatcgcggatcagcatgccgcggtgaatacgttcccgggccttgtacacaccgcccgtcacaccatgagagtcgggaacacccgaagtccgtagcctaaccgcaaggagggcgcggccgaaggtgggttcgataattggggtgaagtcgtaacaaggtagccgt

SEQ ID NO: 59 - DNA, 1511 bp, Clostridium leptum
  rRNA (1)..(1511): 16S rRNA coding gene sequence of Clostridium strain 39
agagtttgatcctggctcaggacgaacgctggcggcgtgcttaacacatgcaagtcgaacggagcacccctgaaggagttttcggacaacggatgggaatgcttagtggcggactggtgagtaacgcgtgaggaacctgccttccagagggggacaacagttggaaacgactgctaataccgcatgatgcgttggagccgcatgactccgacgtcaaagatttatcgctggaagatggcctcgcgtctgattagctagttggtgaggtaacggcccaccaaggcgacgatcagtagccggactgagaggttggccggccacattgggactgagatacggcccagactcctacgggaggcagcagtggggaatattgggcaatggacgcaagtctgacccagcaacgccgcgtgaaggaagaaggctttcgggttgtaaacttcttttaagggggaagagcagaagacggtaccccttgaataagccacggctaactacgtgccagcagccgcggtaatacgtaggtggcaagcgttgtccggatttactgggtgtaaagggcgtgcagccggagagacaagtcagatgtgaaatccacgggctcaacccgtgaactgcatttgaaactgtttcccttgagtgtcggagaggtaatcggaattccttgtgtagcggtgaaatgcgtagatataaggaagacaccagtggcgaagcggattactggacgataactgacggtgaggcgcgaaagcgtggggagcaaacaggattagatacctgggtagtcaacgctgtaaacgatcgatactaggtggtgcgggggacttgaccccctgccgttgccggagttaacaccaataaagtattcggcaccctggggagtacgatcgcaaaggttgaaaactcaaaagaaatggacggggggccccgccccaagcgggtgggattatgttggtttatttcgaaagcaacgcgaagaaccctaacagggcttgacatcctgctaacgaagtagagatacattaggtgcccttcggggaaagtagagacaggtggtgcatggttgtcgtcagctcgtgtcgtgagatgttgggttaagtcccgcaacgagcgcaacccctattgttagttgctacgcaagagcactctagcgagactgccgttgacaaaacggaggaaggcggggacgacgtcaaatcatcatgccccttatgtcctgggctacacacgtaatacaatggcggttaacaaagggatgcaaagccgcgaggcagagcgaaccccaaaaagccgtcccagttcggatcgcaggctgcaacccgcctgcgtgaagtcggaatcgctagtaatcgcggatcagcatgccgcggtgaatacgttcccgggccttgtacacaccgcccgtcacaccatgagagtcgggaacacccgaagtccgtagcctaaccgcaaggagggcgcggccgaaggtgggttcgataattggggtgaagtcgtaacaaggtagccgt

SEQ ID NO: 60 - DNA, 1499 bp, Clostridium leptum
  rRNA (1)..(1499): 16S rRNA coding gene sequence of Clostridium strain 40
agagtttgatcctggctcaggataaacgctggcggcatgcctaacacatgcaagtcgaacggagcgccttggaaggagacttcggtcaacggaagaggaggcttagtggcggacgggtgagtaacgcgtgaggaacctgcctcagagagggggataacacaccgaaaggtgtgctaataccgcataacatatgagaggggcatccctttcatatcaaagatttattgctttgagatggcctcgcgtccaattagctagttggtgaggtaacggcccaccaaggcgacgattggtagccggactgagaggttgaacggccacattgggactgagacacggcccagactcctacgggaggcagcagtggggaatattgcacaatggggggaaccctgatgcagcaatgccgcgtgaaggatgaaggttttcggattgtaaacttcttttgtacgggacgaagaaagtgacggtaccgtaagaataagccacggctaactacgtgccagcagccgcggtaatacgtaggtggcaagcgttatccggatttactgggtgtaaagggcgagtaggcgggattgcaagtcagatgtgaaaactatgggctcaaccgatagagtgcatttgaaactgcagttcttgagtgatggagaggcaggcggaattcccggtgtagcggtggaatgcgtagatatcgggagggaacaccagtggcgaaggcggcctgctggacattaactgacgctgatgcgcgaaagcgtggggagcaaacaggattagataccctggtagtcacgctgtaaacgatgattactaggtgtggggggtactgacccccttcccgtgccggagttaacacaataagtaatccacctggggagtacggccgcaaggttgaaactcaaaggaattgacgggggcccgcacaagcagtggagtatgtggttttaattcgaagcaacgcgaagaaccttaccagggcttgacatggggatgaccgctttagagatagagctttctcttcggagacatcccacacaggtggtgcatggttgtcgtcagctcgtgtcgtgagatgttgggttaagtcccgcaacgagcgcaacccttattgttagttgctacgcaagagcactctagcgagactgccgttgacaaaacggaggaaggtggggacgacgtcaaatcatcatgccctttatgtcctgggctacacacgtactacaatggcggacatacagagggaagcaagacagcgatgtggagcaaatccctaaaagccgtctcagttcagattgcaggctgcaacccgcctgcatgaagtcggaattgctagtaatcgcggatcagcatgccgcggtgaatacgttcccgggccttgtacacaccgcccgtcacaccatgagagtcggaaacacccgaagcctgtagcccaaccgcaaggggggcgcagtcgaaggtgggtctgataattggggtgaagtcgtaacaaaggtagccgt

SEQ ID NO: 61 - DNA, 1512 bp, Clostridium coccoides
  rRNA (1)..(1512): 16S rRNA coding gene sequence of Clostridium strain 41
agagtttgatcctggctcaggatgaacgctggcggcgtgcttaacacatgcaagtcgaacggagatatcattttcgaagcgattagtttactaagagcggagatgttgctatcttagtggcggacgggtgagtaacgcgtgggtaacctgccttgcactgggggataacacttagaaataggtgctaataccgcataacagtaggagacgcatgtcttttacttgaaaactccggtggtgtaagatggacccgcgtctgattagcttgttggcggggtaacggcccaccaaggcaacgatcagtagccggcctgagagggtgaacggccacattgggactgagacacggcccaaactcctacgggaggcagcagtggggaatattggacaatggggggaaccctgatccagcgacgccgcgtgagtgaagaagtatttcggtatgtaaagctctatcagcagggaagaaagaaatgacggtacctgactaagaagccccggctaactacgtgccagcagccgcggtaatacgtagggggcaagcgttatccggatttactgggtgtaaagggagcgtagacggcgatgcaagtctgaagtgaaaggcgggggcccaacccccggactgctttggaaactgtatggctggagtgcaggagaggtaagtggaattcctagtgtagcggtgaaatgcgtagatattaggaggaacaccagtggcgaaagcggcttactggactgtaactgacgttgaggctcgaaagcgtggggagcaaacaagattagatacctggtagtcacgccgtaaacgatgatcaccggtttcggtgggttatggacccatcggttgcgcagcaaacgcagtagtgatccacctggggagtaacgttcgcaagaatgaaacttcaaaggaaatgacgggggacccggcacaagcggtggaggcatgtgtttaattcgaagcaacgcgaagaaccttacccaagtcttgacatcccgtgacgagtgagtaacgtcactttcccttcggggcagcggagacaggtggtgcatggttgtcgtcagctcgtgtcgtgagatgttgggttaagtcccgcaacgagcgcaacccctatccttagtagccagcgagttaggtcgggcactctagggagactgccggggacaacccggaggaaggtggggatgacgtcaaatcatcatgccccttatgatttgggctacacacgtgctacaatggcgtaaacaaagggaagcgagcctgtgaaggtaagcgaatcccagaaataacgtctcagttcggattgtagtctgcaactcgactacatgaagctggaatcgctagtaatcgcggatcagaatgccgcggtgaatacgttcccgggtcttgtacacaccgcccgtcacaccatgggagtcggaaatgcccgaagtctgtgacccaacctgagaaggagggagcagccgaaggcaggtcggatgactggggtgaagtcgtaacaaggtagccgt

SEQ ID NO: 62 - DNA, 17 bp, Artificial
  Artificially synthesized primer sequence
ggtgaatacgttcccgg

SEQ ID NO: 63 - DNA, 22 bp, Artificial
  Artificially synthesized primer sequence
tacggctaccttgttacgactt

SEQ ID NO: 64 - DNA, 20 bp, Artificial
  Artificially synthesized primer sequence
aaatgacggtacctgactaa

SEQ ID NO: 65 - DNA, 22 bp, Artificial
  Artificially synthesized primer sequence
ctttgagtttcattcttgcgaa

SEQ ID NO: 66 - DNA, 16 bp, Artificial
  Artificially synthesized primer sequence
gcacaagcagtggagt

SEQ ID NO: 67 - DNA, 18 bp, Artificial
  Artificially synthesized primer sequence
cttcctccgttttgtcaa

SEQ ID NO: 68 - DNA, 18 bp, Artificial
  Artificially synthesized primer sequence
gagaggaaggtcccccac

SEQ ID NO: 69 - DNA, 19 bp, Artificial
  Artificially synthesized primer sequence
cgctacttggctggttcag